European Patent Application EP 4 215 207 A1, published July 26, 2023. Title: RECOMBINANT NON-PATHOGENIC MAREK'S DISEASE VIRUS CONSTRUCTS ENCODING INFECTIOUS LARYNGOTRACHEITIS VIRUS AND INFECTIOUS BURSAL DISEASE VIRUS ANTIGENS. Applicant: Intervet International BV. Application EP. The sequence listing filed with the application follows.

SEQUENCE LISTING (19 sequences)

SEQ ID NO: 1 - DNA, 1134 bp, Infectious laryngotracheitis virus
  source 1..1134: mol_type = genomic DNA
atggaccgccatttatttttgaggaatgctttttggactatcgtactgctttcttccttcgctagccagagcaccgccgccgtcacgtacgactacattttaggccgtcgcgcgctcgacgcgctaaccataccggcggttggcccgtataacagatacctcactagggtatcaagaggctgcgacgttgtcgagctcaacccgatttctaacgtggacgacatgatatcggcggccaaagaaaaagagaaggggggccctttcgaggcctccgtcgtctggttctacgtgattaagggcgacgacggcgaggacaagtactgtccaatctatagaaaagagtacagggaatgtggcgacgtacaactgctatctgaatgcgccgttcaatctgcacagatgtgggcagtggactatgttcctagcacccttgtatcgcgaaatggcgcgggactgactatattctcccccactgctgcgctctctggccaatacttgctgaccctgaaaatcgggagatttgcgcaaacagctctcgtaactctagaagttaacgatcgctgtttaaagatcgggtcgcagcttaactttttaccgtcgaaatgctggacaacagaacagtatcagactggatttcaaggcgaacacctttatccgatcgcagacaccaatacacgacacgcggacgacgtatatcggggatacgaagatattctgcagcgctggaataatttgctgaggaaaaagaatcctagcgcgccagaccctcgtccagatagcgtcccgcaagaaattcccgctgtaaccaagaaagcggaagggcgcaccccggacgcagaaagcagcgaaaagaaggcccctccagaagactcggaggacgacatgcaggcagaggcttctggagaaaatcctgccgccctccccgaagacgacgaagtccccgaggacaccgagcacgatgatccaaactcggatcctgactattacaatgacatgcccgccgtgatcccggtggaggagactactaaaagttctaatgccgtctccatgcccatattcgcggcgttcgtagcctgcgcggtcgcgctcgtggggctactggtttggagcatcgtaaaatgcgcgcgtagctaa

SEQ ID NO: 2 - protein, 377 aa, Infectious laryngotracheitis virus
MDRHLFLRNAFWTIVLLSSFASQSTAAVTYDYILGRRALDALTIPAVGPYNRYLTRVSRGCDVVELNPISNVDDMISAAKEKEKGGPFEASVVWFYVIKGDDGEDKYCPIYRKEYRECGDVQLLSECAVQSAQMWAVDYVPSTLVSRNGAGLTIFSPTAALSGQYLLTLKIGRFAQTALVTLEVNDRCLKIGSQLNFLPSKCWTTEQYQTGFQGEHLYPIADTNTRHADDVYRGYEDILQRWNNLLRKKNPSAPDPRPDSVPQEIPAVTKKAEGRTPDAESSEKKAPPEDSEDDMQAEASGENPAALPEDDEVPEDTEHDDPNSDPDYYNDMPAVIPVEETTKSSNAVSMPIFAAFVACAVALVGLLVWSIVKCARS

SEQ ID NO: 3 - DNA, 1089 bp, Infectious laryngotracheitis virus
  source 1..1089: mol_type = genomic DNA
atggcatcgctacttggaactctggctctccttgccgcgacgctcgcacccttcggcgcgatgggaatcgtgatcactggaaatcacgtctccgccaggattgacgacgatcacatcgtgatcgtcgcgcctcgccccgaagctacaattcaactgcagctatttttcatgcctggccagagaccccacaaaccctactcaggaaccgtccgcgtcgcgtttcggtctgatataacaaaccagtgctaccaggaacttagcgaggagcgctttgaaaattgcactcatcgatcgtcttctgtttttgtcggctgtaaagtgaccgagtacacgttctccgcctcgaacagactaaccggacctccacacccgtttaagctcactatacgaaatcctcgtccgaacgacagcgggatgttctacgtaattgttcggctagacgacaccaaagaacccattgacgtcttcgcgatccaactatcggtgtatcaattcgcgaacaccgccgcgactcgcggactctattccaaggcttcgtgtcgcaccttcggattacctaccgtccaacttgaggcctatctcaggaccgaggaaagttggcgcaactggcaagcgtacgttgccacggaggccacgacgaccagcgccgaggcgacaaccccgacgcccgtcactgcaaccagcgcctccgaacttgaagcggaacactttacctttccctggctagaaaatggcgtggatcattacgaaccgacacccgcaaacgaaaattcaaacgttactgtccgtctcgggacaatgagccctacgctaattggggtaaccgtggctgccgtcgtgagcgcaacgatcggcctcgtcattgtaatttccatcgtcaccagaaacatgtgcaccccgcaccgaaaattagacacggtctcgcaagacgacgaagaacgttcccaaactagaagggaatcgcgaaaatttggacccatggttgcgtgcgaaataaacaagggggctgaccaggatagtgaacttgtggaactggttgcgattgttaacccgtctgcgctaagctcgcccgactcaataaaaatgtga

SEQ ID NO: 4 - protein, 362 aa, Infectious laryngotracheitis virus
MASLLGTLALLAATLAPFGAMGIVITGNHVSARIDDDHIVIVAPRPEATIQLQLFFMPGQRPHKPYSGTVRVAFRSDITNQCYQELSEERFENCTHRSSSVFVGCKVTEYTFSASNRLTGPPHPFKLTIRNPRPNDSGMFYVIVRLDDTKEPIDVFAIQLSVYQFANTAATRGLYSKASCRTFGLPTVQLEAYLRTEESWRNWQAYVATEATTTSAEATTPTPVTATSASELEAEHFTFPWLENGVDHYEPTPANENSNVTVRLGTMSPTLIGVTVAAVVSATIGLVIVISIVTRNMCTPHRKLDTVSQDDEERSQTRRESRKFGPMVACEINKGADQDSELVELVAIVNPSALSSPDSIKM

SEQ ID NO: 5 - DNA, 1362 bp, Infectious bursal disease virus
  source 1..1362: mol_type = genomic DNA
atgacaaacctgcaagatcaaacccaacagattgttccgttcatacggagccttctgatgccaacaaccggaccggcgtccattccggacgacaccctggagaagcacactctcaggtcagagacctcgacctacaatttgactgtgggggacacagggtcagggctaattgtctttttccctggattccctggctcaattgtgggtgctcactacacactgcagagcaatgggaactacaagttcgatcagatgctcctgactgcccagaacctaccggccagctacaactactgcagactagtgagtcggagtctcacagtgaggtcaagcacactccctggtggcgtttatgcactaaacggcaccataaacgccgtgaccttccaaggaagcctgagtgaactgacagatgttagctacaatgggttgatgtctgcaacagccaacatcaacgacaaaattgggaatgtcctggtaggggaaggggtcactgtcctcagcctacccacatcatatgatcttgggtatgtgaggcttggtgaccccattcccgctatagggcttgacccaaaaatggtagctacatgcgacagcagtgacaggcccagagtctacaccataactgcagccgatgattaccaattctcatcacagtaccaaccaggtggggtaacaatcacactgttctcagccaacattgatgctatcacaagcctcagcattgggggagagctcgtgtttcaaacaagcgtccaaggccttgtactgggcgccaccatctaccttataggctttgatgggactgcggtaatcaccagagctgtggccgcagataatgggctgacggccggcaccgacaatcttatgccattcaatcttgtcattccaaccaatgagataacccagccaatcacatccatcaaactggagatagtgacctccaaaagtggtggtcaggcaggggatcagatgtcatggtcggcaagtgggagcctagcagtgacgatccatggtggcaactatccaggggccctccgtcccgtcacactagtagcctacgaaagagtggcaacaggatccgtcgttacggtcgctggggtgagtaacttcgagctgattccaaatcctgaactagcaaagaacctggttacagaatacggccgatttgacccaggagccatgaactacacaaaattgatactgagtgagagggaccgtcttggcatcaagaccgtctggccaacaagggagtacactgattttcgtgagtacttcatggaggtggccgacctcaactctcccctgaagattgcaggagcatttggcttcaaagacataatccgggctataaggaggtaa

SEQ ID NO: 6 - protein, 453 aa, Infectious bursal disease virus
MTNLQDQTQQIVPFIRSLLMPTTGPASIPDDTLEKHTLRSETSTYNLTVGDTGSGLIVFFPGFPGSIVGAHYTLQSNGNYKFDQMLLTAQNLPASYNYCRLVSRSLTVRSSTLPGGVYALNGTINAVTFQGSLSELTDVSYNGLMSATANINDKIGNVLVGEGVTVLSLPTSYDLGYVRLGDPIPAIGLDPKMVATCDSSDRPRVYTITAADDYQFSSQYQPGGVTITLFSANIDAITSLSIGGELVFQTSVQGLVLGATIYLIGFDGTAVITRAVAADNGLTAGTDNLMPFNLVIPTNEITQPITSIKLEIVTSKSGGQAGDQMSWSASGSLAVTIHGGNYPGALRPVTLVAYERVATGSVVTVAGVSNFELIPNPELAKNLVTEYGRFDPGAMNYTKLILSERDRLGIKTVWPTREYTDFREYFMEVADLNSPLKIAGAFGFKDIIRAIRR

SEQ ID NO: 7 - DNA, 527 bp, Infectious laryngotracheitis virus
  source 1..527: mol_type = genomic DNA
aaacagctgtactacagagtaaccgatggaagaacatcggtccagctaatgtgcctgtcgtgcacgagccattctccggaaccttactgtcttttcgacacgtctcttatagcgagggaaaaagatatcgcgccagagttatactttacctctgatccgcaaacggcatactgcacaataactctgccgtccggcgttgttccgagattcgaatggagccttaataatgtttcactgccggaatatttgacggccacgaccgttgtttcgcataccgctggccaaagtacagtgtggaagagcagcgcgagagcaggcgaggcgtggatttctggccggggaggcaatatatacgaatgcaccgtcctcatctcagacggcactcgcgttactacgcgaaaggagaggtgcttaacaaacacatggattgcggtggaaaacggtgctgctcaggcgcagctgtattcactcttttctggacttgtgtcaggattatgcgggagcatatctgctttgtacgcaacgct

SEQ ID NO: 8 - DNA, 264 bp, Infectious laryngotracheitis virus
  source 1..264: mol_type = genomic DNA
tgactattacaatgacatgcccgccgtgatcccggtggaggagactactaaaagttctaatgccgtctccatgcccatattcgcggcgttcgtagcctgcgcggtcgcgctcgtggggctactggtttggagcatcgtaaaatgcgcgcgtagctaatcgagcctagaataggtggtttcttcctacatgccacgcctcacgctcataatataaatcacatggaatagcataccaatgcctattcattgggacgttcgaaaagc

SEQ ID NO: 9 - DNA, 3563 bp, Infectious laryngotracheitis virus
  source 1..3563: mol_type = genomic DNA
tcgacggcagagtcgcagacgcccctattggacgtcaaaattgtagaggtgaagttttcaaacgatggcgaagtaacggcgacttgcgtttccaccgtcaaatctccctatagggtagaaactaattggaaagtagacctcgtagatgtaatggatgaaatttctgggaacagtcccgccggggtttttaacagtaatgagaaatggcagaaacagctgtactacagagtaaccgatggaagaacatcggtccagctaatgtgcctgtcgtgcacgagccattctccggaaccttactgtcttttcgacacgtctcttatagcgagggaaaaagatatcgcgccagagttatactttacctctgatccgcaaacggcatactgcacaataactctgccgtccggcgttgttccgagattcgaatggagccttaataatgtttcactgccggaatatttgacggccacgaccgttgtttcgcataccgctggccaaagtacagtgtggaagagcagcgcgagagcaggcgaggcgtggatttctggccggggaggcaatatatacgaatgcaccgtcctcatctcagacggcactcgcgttactacgcgaaaggagaggtgcttaacaaacacatggattgcggtggaaaacggtgctgctcaggcgcagctgtattcactcttttctggacttgtgtcaggattatgcgggagcatatctgctttgtacgcaacgctatggaccgccatttatttttgaggaatgctttttggactatcgtactgctttcttccttcgctagccagagcaccgccgccgtcacgtacgactacattttaggccgtcgcgcgctcgacgcgctaaccataccggcggttggcccgtataacagatacctcactagggtatcaagaggctgcgacgttgtcgagctcaacccgatttctaacgtggacgacatgatatcggcggccaaagaaaaagagaaggggggccctttcgaggcctccgtcgtctggttctacgtgattaagggcgacgacggcgaggacaagtactgtccaatctatagaaaagagtacagggaatgtggcgacgtacaactgctatctgaatgcgccgttcaatctgcacagatgtgggcagtggactatgttcctagcacccttgtatcgcgaaatggcgcgggactgactatattctcccccactgctgcgctctctggccaatacttgctgaccctgaaaatcgggagatttgcgcaaacagctctcgtaactctagaagttaacgatcgctgtttaaagatcgggtcgcagcttaactttttaccgtcgaaatgctggacaacagaacagtatcagactggatttcaaggcgaacacctttatccgatcgcagacaccaatacacgacacgcggacgacgtatatcggggatacgaagatattctgcagcgctggaataatttgctgaggaaaaagaatcctagcgcgccagaccctcgtccagatagcgtcccgcaagaaattcccgctgtaaccaagaaagcggaagggcgcaccccggacgcagaaagcagcgaaaagaaggcccctccagaagactcggaggacgacatgcaggcagaggcttctggagaaaatcctgccgccctccccgaagacgacgaagtccccgaggacaccgagcacgatgatccaaactcggatcctgactattacaatgacatgcccgccgtgatcccggtggaggagactactaaaagttctaatgccgtctccatgcccatattcgcggcgttcgtagcctgcgcggtcgcgctcgtggggctactggtttggagcatcgtaaaatgcgcgcgtagctaatcgagcctagaataggtggtttcttcctacatgccacgcctcacgctcataatataaatcacatggaatagcataccaatgcctattcattgggacgttcgaaaagcatggcatcgctacttggaactctggctctccttgccgcgacgctcgcacccttcggcgcgatgggaatcgtgatcactggaaatcacgtctccgccaggattgacgacgatcacatcgtgatcgtcgcgcctcgccccgaagctacaattcaactgcagctatttttcatgcctggccagagaccccacaaaccctactcaggaaccgtccgcgtcgcgtttcggtctgatataacaaaccagtgctaccaggaacttagcgaggagcgctttgaaaattgcactcatcgatcgtcttctgtttttgtcggctgtaaagtgaccgagtacacgttctccgcctcgaacagactaaccggacctccacacccgtttaagctcactatacgaaatcctcgtccgaacgacagcgggatgttctacgtaattgttcggctagacgacaccaaagaacccattgacgtcttcgcgatccaactatcggtgtatcaattcgcgaacaccgccgcgactcgcggactctattccaaggcttcgtgtcgcaccttcggattacctaccgtccaacttgaggcctatctcaggaccgaggaaagttggcgcaactggcaagcgtacgttgccacggaggccacgacgaccagcgccgaggcgacaaccccgacgcccgtcactgcaaccagcgcctccgaacttgaagcggaacactttacctttccctggctagaaaatggcgtggatcattacgaaccgacacccgcaaacgaaaattcaaacgttactgtccgtctcgggacaatgagccctacgctaattggggtaaccgtggctgccgtcgtgagcgcaacgatcggcctcgtcattgtaatttccatcgtcaccagaaacatgtgcaccccgcaccgaaaattagacacggtctcgcaagacgacgaagaacgttcccaaactagaagggaatcgcgaaaatttggacccatggttgcgtgcgaaataaacaagggggctgaccaggatagtgaacttgtggaactggttgcgattgttaacccgtctgcgctaagctcgcccgactcaataaaaatgtgattaagtctgaatgtggctctccaatcatttcgattctctaatctcccaatcctctcaaaaggggcagtatcggacacggactgggaggggcgtacacgatagttatatggtacagcagaggcctctgaacacttaggaggagaattcagccggggagagcccctgttgagtaggcttgggagcatattgcaggatgaacatgttagtgatagttctcgcctcttgtcttgcgcgcctaacttttgcgacgcgacacgtcctctttttggaaggcactcaggctgtcctcggggaagatgatcccagaaacgttccggaagggactgtaatcaaatggacaaaagtcctgcggaacgcgtgcaagatgaaggcggccgatgtctgctcttcgcctaactattgctttcatgatttaatttacgacggaggaaagaaagactgcccgcccgcgggacccctgtctgcaaacctggtaattttactaaagcgcggcgaa

SEQ ID NO: 10 - DNA, 1391 bp, Murine cytomegalovirus
  source 1..1391: mol_type = genomic DNA
aactccgcccgttttatgactagaaccaatagtttttaatgccaaatgcactgaaatcccctaatttgcaaagccaaacgccccctatgtgagtaatacggggactttttacccaatttcccacgcggaaagccccctaatacactcatatggcatatgaatcagcacggtcatgcactctaatggcggcccatagggactttccacatagggggcgttcaccatttcccagcataggggtggtgactcaatggcctttacccaagtacattgggtcaatgggaggtaagccaatgggtttttcccattactggcaagcacactgagtcaaatgggactttccactgggttttgcccaagtacattgggtcaatgggaggtgagccaatgggaaaaacccattgctgccaagtacactgactcaatagggactttccaatgggtttttccattgttggcaagcatataaggtcaatgtgggtgagtcaatagggactttccattgtattctgcccagtacataaggtcaatagggggtgaatcaacaggaaagtcccattggagccaagtacactgcgtcaatagggactttccattgggttttgcccagtacataaggtcaataggggatgagtcaatgggaaaaacccattggagccaagtacactgactcaatagggactttccattgggttttgcccagtacataaggtcaatagggggtgagtcaacaggaaagttccattggagccaagtacattgagtcaatagggactttccaatgggttttgcccagtacataaggtcaatgggaggtaagccaatgggtttttcccattactggcacgtatactgagtcattagggactttccaatgggttttgcccagtacataaggtcaataggggtgaatcaacaggaaagtcccattggagccaagtacactgagtcaatagggactttccattgggttttgcccagtacaaaaggtcaatagggggtgagtcaatgggtttttcccattattggcacgtacataaggtcaataggggtgagtcattgggtttttccagccaatttaattaaaacgccatgtactttcccaccattgacgtcaatgggctattgaaactaatgcaacgtgacctttaaacggtactttcccatagctgattaatgggaaagtaccgttctcgagccaatacacgtcaatgggaagtgaaagggcagccaaaacgtaacaccgccccggttttcccctggaaattccatattggcacgcattctattggctgagctgcgttctacgtgggtataagaggcgcgaccagcgtcggtaccgtcgcagtcttcggtctgaccaccgtagaacgcagagctcctcgctgcag

SEQ ID NO: 11 - DNA, 692 bp, Gallus gallus
  misc_feature 141..143: note = n is a, c, g, or t
  source 1..692: mol_type = genomic DNA
cgcgccggatcagatctccatggtcgaggtgagccccacgttctgcttcactctccccatctcccccccctccccacccccaattttgtatttatttattttttaattattttgtgcagcgatgggggcgggggggggggnnncgcgcgccaggcggggcggggcggggcgaggggcggggcggggcgaggcggagaggtgcggcggcagccaatcagagcggcgcgctccgaaagtttccttttatggcgaggcggcggcggcggcggccctataaaaagcgaagcgcgcggcgggcgggagtcgctgcgcgctgccttcgccccgtgccccgctccgccgccgcctcgcgccgcccgccccggctctgactgaccgcgttactcccacaggtgagcgggcgggacggcccttctcctccgggctgtaattagcggcaggaaggaaatgggcggggagggccttcgtgcgtcgccgcgccgccgtccccttctccctctccagcctcggggctgtccgcggggggacggctgccttcgggggggacggggcagggcggggttcggcttctggcgtgtgaccggcggctctagagcctctgctaaccatgttcatgccttcttctttttcctacagctcctgggcaacgtgctggttattgtgctgtctcatcattttggcaaagaattgca

SEQ ID NO: 12 - DNA, 301 bp, Human cytomegalovirus
  source 1..301: mol_type = genomic DNA
ggcagtacatctacgtattagtcatcgctattaccatggtgatgcggttttggcagtacatcaatgggcgtggatagcggtttgactcacggggatttccaagtctccaccccattgacgtcaatgggagtttgttttggcaccaaaatcaacgggactttccaaaatgtcgtaacaactccgccccattgacgcaaatgggcggtaggcgtgtacggtgggaggtctatataagcagagctcgtttagtgaaccgtcagatcgcctggagacgccatccacgctgttttgacctccatag

SEQ ID NO: 13 - DNA, 55 bp, Feline herpesvirus
  source 1..55: mol_type = genomic DNA
caataaacatagcatacgttatgacatggtctaccgcgtcttatatggggacgac

SEQ ID NO: 14 - DNA, 370 bp, Herpes simplex virus
  source 1..370: mol_type = genomic DNA
gatccataattgattgacgggagatgggggaggctaactgaaacacggaaggagacaataccggaaggaacccgcgctatgacggcaataaaaagacagaataaaacgcacgggtgttgggtcgtttgttcataaacgcggggttcggtcccagggctggcactctgtcgataccccaccgagaccccattggggccaatacgcccgcgtttcttccttttccccaccccaccccccaagttcgggtgaaggcccagggctcgcagccaacgtcggggcggcaggccctgccatagccactggccccgtgggttagggacggggtcccccatggggaatggtttatggttcgtgggggttattattttga

SEQ ID NO: 15 - DNA, 14113 bp, synthetic construct
  misc_feature 1..14113: note = Herpesvirus of turkeys, Murine cytomegalovirus, Infectious bursal disease virus, Simian vacuolating virus 40, and Infectious laryngotracheitis virus
  source 1..14113: mol_type = other DNA
gaattccagactaaatgccccggcccaatttgtcaagtgtgcagtcacggaggcgtcgaccgtgtccccggcattaaacaggaaagcgttaaagtttttgaatgttaggtcacaggtacaaacataaatgtttgtacaaacaggtaacaggtacaaacataaatgccccggcataaatgtcccttacggcggatcgaaacgacattaggcatactcgggtaccattttgcattccgatcagcacggatgaaattaggcaggaatgcggtttatattatgcggcattggacaaacgatatggcattgattggcagtttatgaatgtcttcatgttgggcgtaaacggattcctattggttcagaagacaacgacgatatatttagagagaaaaagctacccagcataggataaacacacattgagcattgagagacataggtatcggtatggatgggaaaactacacacgtgaacaccaaacgacttatatactcgagcggtgatactactgagcaagaatgcactgcatctgagccactgaatgaagactgtgatgaaaatgtgaccatcgatggaattggagaagaatatgcgcagttcttcatgtccccgcaatgggtcccaaatctacatcgcttgagcgaggataccaaaaaggtataccgatgtatggtttccaacagactcaattattttccctattatgaggcgttcaggcggtctttgtttgatatgtatatgctaggtcggttggggcgtcgacttaagcgatctgactgggagactattatgcatctgtcaccaacgcaaagtcggcgtctacatagaactttaagatttgtggagcgtagaattatcccatctaacagttatatacgcacatcgggccacgttccgccttcgagggcacttccgacagatacgaatttaaagatggatgaataattaaattggaaagagtaactacattaatcgagcgtcatgacggcgtcccgtgaaaatgggaattttctactcgaaacaccgtgacatttgacagacctggaattgttattctgatatatagtgggtgtgtctggccggcaacatacataatgtgcatgcgaaaccactttttcagtgtacgctgacattgtgcaacacggaggggtagcatctacatacaatatatgttgattaatgattggagaaaaaactatgcagctcgccgatcatatggctaactcgccttcgtctatatggcggaccccgcgggaaaaatcgacgtaccatctgatttacaacaccagtaatgaacatgtcgcatccctgcccagatctgtgcgcccattggcgcggatcgttgtgaatgccgccgaaacacttcaggtcggtatgagagccgggaggccgccatcagcaggagtttggcgagaggtgtttgatagaatgatgacagccttccgtgaccacgagcctactgcgacatttaatgctgcaaatcccattagaaaaatggtcgagacagttctacagaataatgaagagcccccgcggacgcatgctgaaatgggtaatcgccttatgaacattatgtactggtgttgcttgggacacgcaggacaatgctcgatatggcagttgtacgagacgaatcaggccattttaagtttattagatgaagtggttatcggcacaacaaatcccttttgcaccctcgagcaatactggaagccattatgcaccgcaatcgccaacaaggggacctcatcgcttgttgaggatgccaaagtggccgagtacctggttagcatgcgcaaattgatataacataggcacgctctgatgttacagaccacaataccgcatacatttattgtaaggttgttaataaaggtttattctatgtaagactacaatactttcgacattgcttgtatacatattaaatactttctcaagttcctattacataaaatgggatctatcattacattcgttaagagtctggataattttactgtttgccagcttcgatcttggaacgtactgtggatagtgccttacttggaatcgtgaaaatttgaaacgtccattatttggatatcttccggttgtcccatatcccgccctggtaccgctcggataccttgcccgtatggattcgtattgacagtcgcgcaatcggggaccaacaacgcgtgggtccacactcattcggaaattttccgatgattctgaatatttattgccgctcgttacgagtcgttggacatatctgtaatacatttcttcttctgaaggatcgctgcacatttgatctatacattggccaggatgttcaagtctcagatgttgcattctggcacagcacaactttatggcatttccgatgtaatcgtccggcagccctgggggagttctatattcgcatattgggatggtaaggacaatagcagatctcgcaacctccagggaggctataataacgtttttaaaggatggatttctcataaaaatctgtcgcaaattacactgagaatatcctttactagcgccgattgagagcatcgtcgtccaattttctaaatggaaagaaaacaaggcgggcaagagtgttccaaacattttcattttcggcgaatctctcaaatcccatggcgtgcaattgattgcaaaattggcacttccgttcacgtttgtatctccaaactctaagacacttttaattgaaaaactacgttctagtgtggaaagaaacctataggcagaccatagaactatttgacaccacatatctttttgtatgtcaaactgaccatgatcgtatgttgctgaatgcactagggcaattcgctcgcgcgactccatacattgaataattccacacgtcagctcatcggttagcaaggtccagtagttgaagtcatttatttttccccgcggctggccaaatctacctctgggaatatccaagttgtcgaatatgatcgcaccggctctggtcatggtgaaggaactgtagcataaagacgcaggtatcataggggtaatatttttttattcactcacatactaaaagtaacgcatattagcaccatgtatgggctatcaattgacatttgcgtagcactacatcacgattatgtacaacataatgggacaacatatggcaagtagatgcaatttcctcacactagttgggtttatctactattgaattttcccctatctgtgatacacttgggagcctctacaagcatattgccatcatgtacgtttttatctactgtcttaacgcccatgggaacggaggcgtcgtcgtcatgtattggacggcaacataggcagcaacacaaattgcgtttaggtggggtgcatgtggactcgataccaagcccctgcagctggggaacgtctggtggagagccgataatttgatatacgcacgccatattactgtcgttgaagtacgccttatcttctatgttttcaaatttaggttcccaagtggacgtgagaagtgtttgtatctcacatggaatggcccaaggcattccagcccaggtgcctggtactttaatggcaaacaaacgttttggtagaggtattgattctattgcagttctgcagatatctgcagccccgagtatccacaggctatacgatacgttatcggaggcaagctgcggccgctctagaactagtggatcccccgggctgcagcccaatgtggaattcgcccttgcacattgttactcctgcatcttaaaaatatatcctgtagtaattttcacagcaatgtcataacatcatctcgctaaagaatgacctgggattggagaagtaatgaatatttgcaaccaatgcattgaataaactaacattaaacgaattcactagtggatcccccaactccgcccgttttatgactagaaccaatagtttttaatgccaaatgcactgaaatcccctaatttgcaaagccaaacgccccctatgtgagtaatacggggactttttacccaatttcccacgcggaaagccccctaatacactcatatggcatatgaatcagcacggtcatgcactctaatggcggcccatagggactttccacatagggggcgttcaccatttcccagcataggggtggtgactcaatggcctttacccaagtacattgggtcaatgggaggtaagccaatgggtttttcccattactggcaagcacactgagtcaaatgggactttccactgggttttgcccaagtacattgggtcaatgggaggtgagccaatgggaaaaacccattgctgccaagtacactgactcaatagggactttccaatgggtttttccattgttggcaagcatataaggtcaatgtgggtgagtcaatagggactttccattgtattctgcccagtacataaggtcaatagggggtgaatcaacaggaaagtcccattggagccaagtacactgcgtcaatagggactttccattgggttttgcccagtacataaggtcaataggggatgagtcaatgggaaaaacccattggagccaagtacactgactcaatagggactttccattgggttttgcccagtacataaggtcaatagggggtgagtcaacaggaaagttccattggagccaagtacattgagtcaatagggactttccaatgggttttgcccagtacataaggtcaatgggaggtaagccaatgggtttttcccattactggcacgtatactgagtcattagggactttccaatgggttttgcccagtacataaggtcaataggggtgaatcaacaggaaagtcccattggagccaagtacactgagtcaatagggactttccattgggttttgcccagtacaaaaggtcaatagggggtgagtcaatgggtttttcccattattggcacgtacataaggtcaataggggtgagtcattgggtttttccagccaatttaattaaaacgccatgtactttcccaccattgacgtcaatgggctattgaaactaatgcaacgtgacctttaaacggtactttcccatagctgattaatgggaaagtaccgttctcgagccaatacacgtcaatgggaagtgaaagggcagccaaaacgtaacaccgccccggttttcccctggaaattccatattggcacgcattctattggctgagctgcgttctacgtgggtataagaggcgcgaccagcgtcggtaccgtcgcagtcttcggtctgaccaccgtagaacgcagagctcctcgctgcaggcggccgctctagaactcgtcgatcgcagcgatgacaaacctgcaagatcaaacccaacagattgttccgttcatacggagccttctgatgccaacaaccggaccggcgtccattccggacgacaccctggagaagcacactctcaggtcagagacctcgacctacaatttgactgtgggggacacagggtcagggctaattgtctttttccctggattccctggctcaattgtgggtgctcactacacactgcagagcaatgggaactacaagttcgatcagatgctcctgactgcccagaacctaccggccagctacaactactgcagactagtgagtcggagtctcacagtgaggtcaagcacactccctggtggcgtttatgcactaaacggcaccataaacgccgtgaccttccaaggaagcctgagtgaactgacagatgttagctacaatgggttgatgtctgcaacagccaacatcaacgacaaaattgggaatgtcctggtaggggaaggggtcactgtcctcagcctacccacatcatatgatcttgggtatgtgaggcttggtgaccccattcccgctatagggcttgacccaaaaatggtagctacatgcgacagcagtgacaggcccagagtctacaccataactgcagccgatgattaccaattctcatcacagtaccaaccaggtggggtaacaatcacactgttctcagccaacattgatgctatcacaagcctcagcattgggggagagctcgtgtttcaaacaagcgtccaaggccttgtactgggcgccaccatctaccttataggctttgatgggactgcggtaatcaccagagctgtggccgcagataatgggctgacggccggcaccgacaatcttatgccattcaatcttgtcattccaaccaatgagataacccagccaatcacatccatcaaactggagatagtgacctccaaaagtggtggtcaggcaggggatcagatgtcatggtcggcaagtgggagcctagcagtgacgatccatggtggcaactatccaggggccctccgtcccgtcacactagtagcctacgaaagagtggcaacaggatccgtcgttacggtcgctggggtgagtaacttcgagctgattccaaatcctgaactagcaaagaacctggttacagaatacggccgatttgacccaggagccatgaactacacaaaattgatactgagtgagagggaccgtcttggcatcaagaccgtctggccaacaagggagtacactgattttcgtgagtacttcatggaggtggccgacctcaactctcccctgaagattgcaggagcatttggcttcaaagacataatccgggctataaggaggtaagcttcagacatgataagatacattgatgagtttggacaaaccacaactagaatgcagtgaaaaaaatgctttatttgtgaaatttgtgatgctattgctttatttgtaaccattataagctgcaataaacaagttaacaacaacaattgcattcattttatgtttcaggttcagggggaggtgtgggaggttttttcggatcctctagagtcgacggcagagtcgcagacgcccctattggacgtcaaaattgtagaggtgaagttttcaaacgatggcgaagtaacggcgacttgcgtttccaccgtcaaatctccctatagggtagaaactaattggaaagtagacctcgtagatgtaatggatgaaatttctgggaacagtcccgccggggtttttaacagtaatgagaaatggcagaaacagctgtactacagagtaaccgatggaagaacatcggtccagctaatgtgcctgtcgtgcacgagccattctccggaaccttactgtcttttcgacacgtctcttatagcgagggaaaaagatatcgcgccagagttatactttacctctgatccgcaaacggcatactgcacaataactctgccgtccggcgttgttccgagattcgaatggagccttaataatgtttcactgccggaatatttgacggccacgaccgttgtttcgcataccgctggccaaagtacagtgtggaagagcagcgcgagagcaggcgaggcgtggatttctggccggggaggcaatatatacgaatgcaccgtcctcatctcagacggcactcgcgttactacgcgaaaggagaggtgcttaacaaacacatggattgcggtggaaaacggtgctgctcaggcgcagctgtattcactcttttctggacttgtgtcaggattatgcgggagcatatctgctttgtacgcaacgctatggaccgccatttatttttgaggaatgctttttggactatcgtactgctttcttccttcgctagccagagcaccgccgccgtcacgtacgactacattttaggccgtcgcgcgctcgacgcgctaaccataccggcggttggcccgtataacagatacctcactagggtatcaagaggctgcgacgttgtcgagctcaacccgatttctaacgtggacgacatgatatcggcggccaaagaaaaagagaaggggggccctttcgaggcctccgtcgtctggttctacgtgattaagggcgacgacggcgaggacaagtactgtccaatctatagaaaagagtacagggaatgtggcgacgtacaactgctatctgaatgcgccgttcaatctgcacagatgtgggcagtggactatgttcctagcacccttgtatcgcgaaatggcgcgggactgactatattctcccccactgctgcgctctctggccaatacttgctgaccctgaaaatcgggagatttgcgcaaacagctctcgtaactctagaagttaacgatcgctgtttaaagatcgggtcgcagcttaactttttaccgtcgaaatgctggacaacagaacagtatcagactggatttcaaggcgaacacctttatccgatcgcagacaccaatacacgacacgcggacgacgtatatcggggatacgaagatattctgcagcgctggaataatttgctgaggaaaaagaatcctagcgcgccagaccctcgtccagatagcgtcccgcaagaaattcccgctgtaaccaagaaagcggaagggcgcaccccggacgcagaaagcagcgaaaagaaggcccctccagaagactcggaggacgacatgcaggcagaggcttctggagaaaatcctgccgccctccccgaagacgacgaagtccccgaggacaccgagcacgatgatccaaactcggatcctgactattacaatgacatgcccgccgtgatcccggtggaggagactactaaaagttctaatgccgtctccatgcccatattcgcggcgttcgtagcctgcgcggtcgcgctcgtggggctactggtttggagcatcgtaaaatgcgcgcgtagctaatcgagcctagaataggtggtttcttcctacatgccacgcctcacgctcataatataaatcacatggaatagcataccaatgcctattcattgggacgttcgaaaagcatggcatcgctacttggaactctggctctccttgccgcgacgctcgcacccttcggcgcgatgggaatcgtgatcactggaaatcacgtctccgccaggattgacgacgatcacatcgtgatcgtcgcgcctcgccccgaagctacaattcaactgcagctatttttcatgcctggccagagaccccacaaaccctactcaggaaccgtccgcgtcgcgtttcggtctgatataacaaaccagtgctaccaggaacttagcgaggagcgctttgaaaattgcactcatcgatcgtcttctgtttttgtcggctgtaaagtgaccgagtacacgttctccgcctcgaacagactaaccggacctccacacccgtttaagctcactatacgaaatcctcgtccgaacgacagcgggatgttctacgtaattgttcggctagacgacaccaaagaacccattgacgtcttcgcgatccaactatcggtgtatcaattcgcgaacaccgccgcgactcgcggactctattccaaggcttcgtgtcgcaccttcggattacctaccgtccaacttgaggcctatctcaggaccgaggaaagttggcgcaactggcaagcgtacgttgccacggaggccacgacgaccagcgccgaggcgacaaccccgacgcccgtcactgcaaccagcgcctccgaacttgaagcggaacactttacctttccctggctagaaaatggcgtggatcattacgaaccgacacccgcaaacgaaaattcaaacgttactgtccgtctcgggacaatgagccctacgctaattggggtaaccgtggctgccgtcgtgagcgcaacgatcggcctcgtcattgtaatttccatcgtcaccagaaacatgtgcaccccgcaccgaaaattagacacggtctcgcaagacgacgaagaacgttcccaaactagaagggaatcgcgaaaatttggacccatggttgcgtgcgaaataaacaagggggctgaccaggatagtgaacttgtggaactggttgcgattgttaacccgtctgcgctaagctcgcccgactcaataaaaatgtgattaagtctgaatgtggctctccaatcatttcgattctctaatctcccaatcctctcaaaaggggcagtatcggacacggactgggaggggcgtacacgatagttatatggtacagcagaggcctctgaacacttaggaggagaattcagccggggagagcccctgttgagtaggcttgggagcatattgcaggatgaacatgttagtgatagttctcgcctcttgtcttgcgcgcctaacttttgcgacgcgacacgtcctctttttggaaggcactcaggctgtcctcggggaagatgatcccagaaacgttccggaagggactgtaatcaaatggacaaaagtcctgcggaacgcgtgcaagatgaaggcggccgatgtctgctcttcgcctaactattgctttcatgatttaatttacgacggaggaaagaaagactgcccgcccgcgggacccctgtctgcaaacctggtaattttactaaagcgcggcgaagcttagcttgcctccgattctagcattacatagccggtcagtagatcctgccattcggtagcgcaaccggctacatcttcaaacagtctcacgataaatgcatctctcgttcctgccaatccggaaccgggcataccactcccgcctgccgatttaattctcacaattgggcgatgccggcggggcaaaacgaatgtggatttggcaaaccgacacaggtctgctgtacggactaatatgggcacacccacatcattcttcagatgctccatgcattgttctatgagaaagatccatagggtggaggcagcgtcacgagatcgcccaggcaatcgatcgcattcgtctagtaaagtgacgagagttatcatgcacacacccatgcccacgccttccgaataactggagctgtggaagatcggaaacgtctttttgactgccggtctcgtactactttcgcacaggtgtatacccggacgcgtactatatattttatatcatccaacgtccgaaattacatacgtggcggcgatggaagtagatgttgagtcttcgaaagtaagtgcctcgaatatgggtattgtctgtgaaaatatcgaaagcggtacgacggttgcagaaccgtcgatgtcgccagatactagtaacaatagcttcgataacgaagacttccgtgggcctgaatacgatgtggagataaataccagaaaatctgctaatcttgatcgtatggaatcttcgtgccgtgaacaacgagcggcgtgcgaacttcgaaagtgttcgtgtcctacgtctgccgtgcgcatgcaatacagtattctttcatctctcgctccgggttcagagggtcatgtatatatatgtactagatacggggacgcggaccaaaaaaaatgcatagtgaaggcagtcgttggaggaaagaatcccgggagggaagtggatattttaaaaaccatctcacataaatcaattataaaattaatccatgcctataaatggaaaaatgttgtgtgtatggcaatgcgtgtatatcgttatgatcttttcacatatattgacggagtcggccctatgccccttcaacagatgatctatattcaacgtggactactagaggcgctagcatacatacatgaaaggggcatcattcaccgagacgtaaagacggagaatatattcttggataatcacgaaaatgcagttttgggtgacttcggtgctgcatgccaactaggagattgtatagatacgccccaatgttacggttggagcggaactgtggaaacaaattcgccggaattatctgcacttgatccgtattgcacaaaaacagatatttggagtgccggattggttctatatgagatggcaattaaaaatgtaccattgtttagtaagcaggtgaaaagttcgggatctcagctgagatccataatacggtgcatgcaagtgcatgaactggagtttccccgcaacgattctaccaacctctgtaaacatttcaaacaatatgcggttcgtgtacgaccgccttataccattcctcgagttataagaaatggggggatgccaatggatgttgaatatgtcatttctaaaatgcttacgtttgaccaggagttcagaccttctgctaaggaaatattgaatatgcccctatttactaaggcgccgattaacctgcttaatatcacaccctctgacagtgtctaacggtatacaggcgggagcgggtcgtggcgtcatcatcaccacttgagaatttatattttgaattgttgattgataaattaacctgattcattgagaactgaaacgccatattggtttcttggatatgtctacaacaattagttaaattgctatgttctactgcgagtaacatttgataagttgtaagagacgggcgactcatgtcgaagttgacgaatataaagtacataacgtgtttagaatacccagaatccgaatagtccgcgggggcgtcttctcgcgtgagtaccaaatactgagttgaacttgaaaatgctaaatctgtgacactctttgtgtgatgattattgtcaccacttcgaagatggcttcgacattcatgatgttctggtgtttgtttggaatcgtaatagcgcttgtttcgtccaagtctgacaacaaagaaaatctgaagaattatatcacggataagtcaaccaatattagaatacccacgccattatttgtatcaacggaaaactcttatcccacaaaacatgtaatctacgatgaaaactgtggcttcgctgtactcaatcctataagtgaccccaaatatgtccttttgagccagcttctaatgggaaggcgcaaatatgatgcgacggtcgcgtggtttgttctcggtaaaatgtgtgccagattaatatatttgcgcgaattttataactgctcgacaaatgagccttttggcacatgttctatgagctctcctggatggtgggacaggcgctacgtctcaaccagtttcatttctcgcgacgaattacagctggtttttgcagcgccgtcccgagaattagatggtttatatacgcgcgtagtagttgtcaacggggactttactacggccgatataatgtttaatgttaaagtggcatgtgccttttcaaagactggaatagaagatgatacattatgcaaaccctttcatttctttgccaatgcaacattgcacaatttaaccatgattagatcggtaactcttcgagcgcacgaaagccatttaaaggaatgggtggcacggagaggtggtaacgtccctgcagtgctacttgagtctaccatgtatcatgcatccaatctgcctagaaatttcagggatttctacataaagtctccagatgattataagtataatcacctagatgggccatctgtaatgctcatcactgacagacctagtgaagatttggatgggaggctcgttcaccaaagtgacatttttactactacaagtcctataaaacaggtccggtatgaagagcatcagtcacatacaaagcagtatcctgtaaacaaaatacaagctataatttttttgatagggttaggctcgttcattggaagcatattcgtagttttggtagtatggattatacgcagatattgcaatggagcgcggagtgggggaacgccccccagtcctcgccggtatgtgtataccaggctatgatcacgtgtgaaacttgggcggacctgtatcatatgtacaccgtccctattcgtttatagccagtacgtgttatctgcacatagaggaacatgtgtcatactgggatcgcatgcatggtatgtgtgactctaatattattctgtatcataataaaaacacagtgcatggtatatagaggatcgctggtaagcactacggtagaccaatcggctcagattgcattctttggcatcgataccgttgttaatttatatggcaaagtcttgttcatgggagatcagtatttggaggaaatatactctggaacgatggaaatactcaaatggaatcaagctaaccgctgctattctattgcgcatgcaacatattacgccgactgtcctataatcagttctacggtattcagaggatgccgggacgccgttgtttatactaggccccacagcagaattc

SEQ ID NO: 16 - DNA, 13064 bp, synthetic construct
  misc_feature 1..13064: note = Herpesvirus of turkeys, Infectious laryngotracheitis virus, Gallus gallus, Infectious bursal disease virus, and Feline Herpesvirus
  misc_feature 7401..7403: note = n is a, c, g, or t
  source 1..13064: mol_type = other DNA
gaattccagactaaatgccccggcccaatttgtcaagtgtgcagtcacggaggcgtcgaccgtgtccccggcattaaacaggaaagcgttaaagtttttgaatgttaggtcacaggtacaaacataaatgtttgtacaaacaggtaacaggtacaaacataaatgccccggcataaatgtcccttacggcggatcgaaacgacattaggcatactcgggtaccattttgcattccgatcagcacggatgaaattaggcaggaatgcggtttatattatgcggcattggacaaacgatatggcattgattggcagtttatgaatgtcttcatgttgggcgtaaacggattcctattggttcagaagacaacgacgatatatttagagagaaaaagctacccagcataggataaacacacattgagcattgagagacataggtatcggtatggatgggaaaactacacacgtgaacaccaaacgacttatatactcgagcggtgatactactgagcaagaatgcactgcatctgagccactgaatgaagactgtgatgaaaatgtgaccatcgatggaattggagaagaatatgcgcagttcttcatgtccccgcaatgggtcccaaatctacatcgcttgagcgaggataccaaaaaggtataccgatgtatggtttccaacagactcaattattttccctattatgaggcgttcaggcggtctttgtttgatatgtatatgctaggtcggttggggcgtcgacttaagcgatctgactgggagactattatgcatctgtcaccaacgcaaagtcggcgtctacatagaactttaagatttgtggagcgtagaattatcccatctaacagttatatacgcacatcgggccacgttccgccttcgagggcacttccgacagatacgaatttaaagatggatgaataattaaattggaaagagtaactacattaatcgagcgtcatgacggcgtcccgtgaaaatgggaattttctactcgaaacaccgtgacatttgacagacctggaattgttattctgatatatagtgggtgtgtctggccggcaacatacataatgtgcatgcgaaaccactttttcagtgtacgctgacattgtgcaacacggaggggtagcatctacatacaatatatgttgattaatgattggagaaaaaactatgcagctcgccgatcatatggctaactcgccttcgtctatatggcggaccccgcgggaaaaatcgacgtaccatctgatttacaacaccagtaatgaacatgtcgcatccctgcccagatctgtgcgcccattggcgcggatcgttgtgaatgccgccgaaacacttcaggtcggtatgagagccgggaggccgccatcagcaggagtttggcgagaggtgtttgatagaatgatgacagccttccgtgaccacgagcctactgcgacatttaatgctgcaaatcccattagaaaaatggtcgagacagttctacagaataatgaagagcccccgcggacgcatgctgaaatgggtaatcgccttatgaacattatgtactggtgttgcttgggacacgcaggacaatgctcgatatggcagttgtacgagacgaatcaggccattttaagtttattagatgaagtggttatcggcacaacaaatcccttttgcaccctcgagcaatactggaagccattatgcaccgcaatcgccaacaaggggacctcatcgcttgttgaggatgccaaagtggccgagtacctggttagcatgcgcaaattgatataacataggcacgctctgatgttacagaccacaataccgcatacatttattgtaaggttgttaataaaggtttattctatgtaagactacaatactttcgacattgcttgtatacatattaaatactttctcaagttcctattacataaaatgggatctatcattacattcgttaagagtctggataattttactgtttgccagcttcgatcttggaacgtactgtggatagtgccttacttggaatcgtgaaaatttgaaacgtccattatttggatatcttccggttgtcccatatcccgccctggtaccgctcggataccttgcccgtatggattcgtattgacagtcgcgcaatcggggaccaacaacgcgtgggtccacactcattcggaaattttccgatgattctgaatatttattgccgctcgttacgagtcgttggacatatctgtaatacatttcttcttctgaaggatcgctgcacatttgatctatacattggccaggatgttcaagtctcagatgttgcattctggcacagcacaactttatggcatttccgatgtaatcgtccggcagccctgggggagttctatattcgcatattgggatggtaaggacaatagcagatctcgcaacctccagggaggctataataacgtttttaaaggatggatttctcataaaaatctgtcgcaaattacactgagaatatcctttactagcgccgattgagagcatcgtcgtccaattttctaaatggaaagaaaacaaggcgggcaagagtgttccaaacattttcattttcggcgaatctctcaaatcccatggcgtgcaattgattgcaaaattggcacttccgttcacgtttgtatctccaaactctaagacacttttaattgaaaaactacgttctagtgtggaaagaaacctataggcagaccatagaactatttgacaccacatatctttttgtatgtcaaactgaccatgatcgtatgttgctgaatgcactagggcaattcgctcgcgcgactccatacattgaataattccacacgtcagctcatcggttagcaaggtccagtagttgaagtcatttatttttccccgcggctggccaaatctacctctgggaatatccaagttgtcgaatatgatcgcaccggctctggtcatggtgaaggaactgtagcataaagacgcaggtatcataggggtaatatttttttattcactcacatactaaaagtaacgcatattagcaccatgtatgggctatcaattgacatttgcgtagcactacatcacgattatgtacaacataatgggacaacatatggcaagtagatgcaatttcctcacactagttgggtttatctactattgaattttcccctatctgtgatacacttgggagcctctacaagcatattgccatcatgtacgtttttatctactgtcttaacgcccatgggaacggaggcgtcgtcgtcatgtattggacggcaacataggcagcaacacaaattgcgtttaggtggggtgcatgtggactcgataccaagcccctgcagctggggaacgtctggtggagagccgataatttgatatacgcacgccatattactgtcgttgaagtacgccttatcttctatgttttcaaatttaggttcccaagtggacgtgagaagtgtttgtatctcacatggaatggcccaaggcattccagcccaggtgcctggtactttaatggcaaacaaacgttttggtagaggtattgattctattgcagttctgcagatatctgcagccccgagtatccacaggctatacgatacgttatcggaggcaagcttaattaagtaccgagctcgaattggcgcgcccgacggcagagtcgcagacgcccctattggacgtcaaaattgtagaggtgaagttttcaaacgatggcgaagtaacggcgacttgcgtttccaccgtcaaatctccctatagggtagaaactaattggaaagtagacctcgtagatgtaatggatgaaatttctgggaacagtcccgccggggtttttaacagtaatgagaaatggcagaaacagctgtactacagagtaaccgatggaagaacatcggtccagctaatgtgcctgtcgtgcacgagccattctccggaaccttactgtcttttcgacacgtctcttatagcgagggaaaaagatatcgcgccagagttatactttacctctgatccgcaaacggcatactgcacaataactctgccgtccggcgttgttccgagattcgaatggagccttaataatgtttcactgccggaatatttgacggccacgaccgttgtttcgcataccgctggccaaagtacagtgtggaagagcagcgcgagagcaggcgaggcgtggatttctggccggggaggcaatatatacgaatgcaccgtcctcatctcagacggcactcgcgttactacgcgaaaggagaggtgcttaacaaacacatggattgcggtggaaaacggtgctgctcaggcgcagctgtattcactcttttctggacttgtgtcaggattatgcgggagcatatctgctttgtacgcaacgctatggaccgccatttatttttgaggaatgctttttggactatcgtactgctttcttccttcgctagccagagcaccgccgccgtcacgtacgactacattttaggccgtcgcgcgctcgacgcgctaaccataccggcggttggcccgtataacagatacctcactagggtatcaagaggctgcgacgttgtcgagctcaacccgatttctaacgtggacgacatgatatcggcggccaaagaaaaagagaaggggggccctttcgaggcctccgtcgtctggttctacgtgattaagggcgacgacggcgaggacaagtactgtccaatctatagaaaagagtacagggaatgtggcgacgtacaactgctatctgaatgcgccgttcaatctgcacagatgtgggcagtggactatgttcctagcacccttgtatcgcgaaatggcgcgggactgactatattctcccccactgctgcgctctctggccaatacttgctgaccctgaaaatcgggagatttgcgcaaacagctctcgtaactctagaagttaacgatcgctgtttaaagatcgggtcgcagcttaactttttaccgtcgaaatgctggacaacagaacagtatcagactggatttcaaggcgaacacctttatccgatcgcagacaccaatacacgacacgcggacgacgtatatcggggatacgaagatattctgcagcgctggaataatttgctgaggaaaaagaatcctagcgcgccagaccctcgtccagatagcgtcccgcaagaaattcccgctgtaaccaagaaagcggaagggcgcaccccggacgcagaaagcagcgaaaagaaggcccctccagaagactcggaggacgacatgcaggcagaggcttctggagaaaatcctgccgccctccccgaagacgacgaagtccccgaggacaccgagcacgatgatccaaactcggatcctgactattacaatgacatgcccgccgtgatcccggtggaggagactactaaaagttctaatgccgtctccatgcccatattcgcggcgttcgtagcctgcgcggtcgcgctcgtggggctactggtttggagcatcgtaaaatgcgcgcgtagctaatcgagcctagaataggtggtttcttcctacatgccacgcctcacgctcataatataaatcacatggaatagcataccaatgcctattcattgggacgttcgaaaagcatggcatcgctacttggaactctggctctccttgccgcgacgctcgcacccttcggcgcgatgggaatcgtgatcactggaaatcacgtctccgccaggattgacgacgatcacatcgtgatcgtcgcgcctcgccccgaagctacaattcaactgcagctatttttcatgcctggccagagaccccacaaaccctactcaggaaccgtccgcgtcgcgtttcggtctgatataacaaaccagtgctaccaggaacttagcgaggagcgctttgaaaattgcactcatcgatcgtcttctgtttttgtcggctgtaaagtgaccgagtacacgttctccgcctcgaacagactaaccggacctccacacccgtttaagctcactatacgaaatcctcgtccgaacgacagcgggatgttctacgtaattgttcggctagacgacaccaaagaacccattgacgtcttcgcgatccaactatcggtgtatcaattcgcgaacaccgccgcgactcgcggactctattccaaggcttcgtgtcgcaccttcggattacctaccgtccaacttgaggcctatctcaggaccgaggaaagttggcgcaactggcaagcgtacgttgccacggaggccacgacgaccagcgccgaggcgacaaccccgacgcccgtcactgcaaccagcgcctccgaacttgaagcggaacactttacctttccctggctagaaaatggcgtggatcattacgaaccgacacccgcaaacgaaaattcaaacgttactgtccgtctcgggacaatgagccctacgctaattggggtaaccgtggctgccgtcgtgagcgcaacgatcggcctcgtcattgtaatttccatcgtcaccagaaacatgtgcaccccgcaccgaaaattagacacggtctcgcaagacgacgaagaacgttcccaaactagaagggaatcgcgaaaatttggacccatggttgcgtgcgaaataaacaagggggctgaccaggatagtgaacttgtggaactggttgcgattgttaacccgtctgcgctaagctcgcccgactcaataaaaatgtgattaagtctgaatgtggctctccaatcatttcgattctctaatctcccaatcctctcaaaaggggcagtatcggacacggactgggaggggcgtacacgatagttatatggtacagcagaggcctctgaacacttaggaggagaattcagccggggagagcccctgttgagtaggcttgggagcatattgcaggatgaacatgttagtgatagttctcgcctcttgtcttgcgcgcctaacttttgcgacgcgacacgtcctctttttggaaggcactcaggctgtcctcggggaagatgatcccagaaacgttccggaagggactgtaatcaaatggacaaaagtcctgcggaacgcgtgcaagatgaaggcggccgatgtctgctcttcgcctaactattgctttcatgatttaatttacgacggaggaaagaaagactgcccgcccgcgggacccctgtctgcaaacctggtaattttactaaagcgcggcgggcgcgccggatcagatctccatggtcgaggtgagccccacgttctgcttcactctccccatctcccccccctccccacccccaattttgtatttatttattttttaattattttgtgcagcgatgggggcgggggggggggnnncgcgcgccaggcggggcggggcggggcgaggggcggggcggggcgaggcggagaggtgcggcggcagccaatcagagcggcgcgctccgaaagtttccttttatggcgaggcggcggcggcggcggccctataaaaagcgaagcgcgcggcgggcgggagtcgctgcgcgctgccttcgccccgtgccccgctccgccgccgcctcgcgccgcccgccccggctctgactgaccgcgttactcccacaggtgagcgggcgggacggcccttctcctccgggctgtaattagcggcaggaaggaaatgggcggggagggccttcgtgcgtcgccgcgccgccgtccccttctccctctccagcctcggggctgtccgcggggggacggctgccttcgggggggacggggcagggcggggttcggcttctggcgtgtgaccggcggctctagagcctctgctaaccatgttcatgccttcttctttttcctacagctcctgggcaacgtgctggttattgtgctgtctcatcattttggcaaagaattgcagatctggatctatgacaaacctgcaagatcaaacccaacagattgttccgttcatacggagccttctgatgccaacaaccggaccggcgtccattccggacgacaccctggagaagcacactctcaggtcagagacctcgacctacaatttgactgtgggggacacagggtcagggctaattgtctttttccctggattccctggctcaattgtgggtgctcactacacactgcagagcaatgggaactacaagttcgatcagatgctcctgactgcccagaacctaccggccagctacaactactgcagactagtgagtcggagtctcacagtgaggtcaagcacactccctggtggcgtttatgcactaaacggcaccataaacgccgtgaccttccaaggaagcctgagtgaactgacagatgttagctacaatgggttgatgtctgcaacagccaacatcaacgacaaagttgggaatgtcctggtaggggaaggggtcactgtcctcagcctacccacatcatatgatcttgggtatgtgaggcttggtgaccccattcccgctatagggcttgacccaaaaatggtagctacatgcgacagcagtgacaggcccagagtctacaccataactgcagccgatgattaccaattctcatcacagtaccaaccaggtggggtaacaatcacactgttctcagccaacattgatgctatcacaagcctcagcattgggggagagctcgtgtttcaaacaagcgtccaaggccttgtactgggcgccaccatctaccttataggctttgatgggactgcggtaatcaccagagctgtggccgcagataatgggctgacggccggcaccgacaatcttatgccattcaatcttgtcattccaaccaatgagataacccagccgatcacatccatcaaactggagatagtgacctccaaaagtggtggtcaggcaggggatcagatgtcatggtcggcaagtgggagcctagcagtgacgatccatggtggcaactatccaggggccctccgtcccgtcacactagtagcctacgaaagagtggcaacaggatccgtcgttacggtcgctggggtgagtaacttcgagctgatcccaaatcctgaactagcaaagaacctggttacagaatacggccgatttgacccaggagccatgaactacacaaaattgatactgagtgagagggaccgtcttggcatcaagaccgtctggccaacaagggagtacactgattttcgtgagtacttcatggaggtggccgacctcaactctcccctgaagattgcaggagcatttggcttcaaagacataatccgggctataaggaggtaagatccgatctctcgattaattaacaataaacatagcatacgttatgacatggtctaccgcgtcttatatggggacgacaagcttgcctccgattctagcattacatagccggtcagtagatcctgccattcggtagcgcaaccggctacatcttcaaacagtctcacgataaatgcatctctcgttcctgccaatccggaaccgggcataccactcccgcctgccgatttaattctcacaattgggcgatgccggcggggcaaaacgaatgtggatttggcaaaccgacacaggtctgctgtacggactaatatgggcacacccacatcattcttcagatgctccatgcattgttctatgagaaagatccatagggtggaggcagcgtcacgagatcgcccaggcaatcgatcgcattcgtctagtaaagtgacgagagttatcatgcacacacccatgcccacgccttccgaataactggagctgtggaagatcggaaacgtctttttgactgccggtctcgtactactttcgcacaggtgtatacccggacgcgtactatatattttatatcatccaacgtccgaaattacatacgtggcggcgatggaagtagatgttgagtcttcgaaagtaagtgcctcgaatatgggtattgtctgtgaaaatatcgaaagcggtacgacggttgcagaaccgtcgatgtcgccagatactagtaacaatagcttcgataacgaagacttccgtgggcctgaatacgatgtggagataaataccagaaaatctgctaatcttgatcgtatggaatcttcgtgccgtgaacaacgagcggcgtgcgaacttcgaaagtgttcgtgtcctacgtctgccgtgcgcatgcaatacagtattctttcatctctcgctccgggttcagagggtcatgtatatatatgtactagatacggggacgcggaccaaaaaaaatgcatagtgaaggcagtcgttggaggaaagaatcccgggagggaagtggatattttaaaaaccatctcacataaatcaattataaaattaatccatgcctataaatggaaaaatgttgtgtgtatggcaatgcgtgtatatcgttatgatcttttcacatatattgacggagtcggccctatgccccttcaacagatgatctatattcaacgtggactactagaggcgctagcatacatacatgaaaggggcatcattcaccgagacgtaaagacggagaatatattcttggataatcacgaaaatgcagttttgggtgacttcggtgctgcatgccaactaggagattgtatagatacgccccaatgttacggttggagcggaactgtggaaacaaattcgccggaattatctgcacttgatccgtattgcacaaaaacagatatttggagtgccggattggttctatatgagatggcaattaaaaatgtaccattgtttagtaagcaggtgaaaagttcgggatctcagctgagatccataatacggtgcatgcaagtgcatgaactggagtttccccgcaacgattctaccaacctctgtaaacatttcaaacaatatgcggttcgtgtacgaccgccttataccattcctcgagttataagaaatggggggatgccaatggatgttgaatatgtcatttctaaaatgcttacgtttgaccaggagttcagaccttctgctaaggaaatattgaatatgcccctatttactaaggcgccgattaacctgcttaatatcacaccctctgacagtgtctaacggtatacaggcgggagcgggtcgtggcgtcatcatcaccacttgagaatttatattttgaattgttgattgataaattaacctgattcattgagaactgaaacgccatattggtttcttggatatgtctacaacaattagttaaattgctatgttctactgcgagtaacatttgataagttgtaagagacgggcgactcatgtcgaagttgacgaatataaagtacataacgtgtttagaatacccagaatccgaatagtccgcgggggcgtcttctcgcgtgagtaccaaatactgagttgaacttgaaaatgctaaatctgtgacactctttgtgtgatgattattgtcaccacttcgaagatggcttcgacattcatgatgttctggtgtttgtttggaatcgtaatagcgcttgtttcgtccaagtctgacaacaaagaaaatctgaagaattatatcacggataagtcaaccaatattagaatacccacgccattatttgtatcaacggaaaactcttatcccacaaaacatgtaatctacgatgaaaactgtggcttcgctgtactcaatcctataagtgaccccaaatatgtccttttgagccagcttctaatgggaaggcgcaaatatgatgcgacggtcgcgtggtttgttctcggtaaaatgtgtgccagattaatatatttgcgcgaattttataactgctcgacaaatgagccttttggcacatgttctatgagctctcctggatggtgggacaggcgctacgtctcaaccagtttcatttctcgcgacgaattacagctggtttttgcagcgccgtcccgagaattagatggtttatatacgcgcgtagtagttgtcaacggggactttactacggccgatataatgtttaatgttaaagtggcatgtgccttttcaaagactggaatagaagatgatacattatgcaaaccctttcatttctttgccaatgcaacattgcacaatttaaccatgattagatcggtaactcttcgagcgcacgaaagccatttaaaggaatgggtggcacggagaggtggtaacgtccctgcagtgctacttgagtctaccatgtatcatgcatccaatctgcctagaaatttcagggatttctacataaagtctccagatgattataagtataatcacctagatgggccatctgtaatgctcatcactgacagacctagtgaagatttggatgggaggctcgttcaccaaagtgacatttttactactacaagtcctataaaacaggtccggtatgaagagcatcagtcacatacaaagcagtatcctgtaaacaaaatacaagctataatttttttgatagggttaggctcgttcattggaagcatattcgtagttttggtagtatggattatacgcagatattgcaatggagcgcggagtgggggaacgccccccagtcctcgccggtatgtgtataccaggctatgatcacgtgtgaaacttgggcggacctgtatcatatgtacaccgtccctattcgtttatagccagtacgtgttatctgcacatagaggaacatgtgtcatactgggatcgcatgcatggtatgtgtgactctaatattattctgtatcataataaaaacacagtgcatggtatatagaggatcgctggtaagcactacggtagaccaatcggctcagattgcattctttggcatcgataccgttgttaatttatatggcaaagtcttgttcatgggagatcagtatttggaggaaatatactctggaacgatggaaatactcaaatggaatcaagctaaccgctgctattctattgcgcatgcaacatattacgccgactgtcctataatcagttctacggtattcagaggatgccgggacgccgttgtttatactaggccccacagcagaattc

SEQ ID NO: 17 - DNA, 13017 bp, synthetic construct
  misc_feature 1..13017: note = Herpesvirus of turkeys, Infectious laryngotracheitis virus, human cytomegalovirus, Infectious bursal disease virus, and Herpes simplex virus
  source 1..13017: mol_type = other DNA
gaattccagactaaatgccccggcccaatttgtcaagtgtgcagtcacggaggcgtcgaccgtgtccccggcattaaacaggaaagcgttaaagtttttgaatgttaggtcacaggtacaaacataaatgtttgtacaaacaggtaacaggtacaaacataaatgccccggcataaatgtcccttacggcggatcgaaacgacattaggcatactcgggtaccattttgcattccgatcagcacggatgaaattaggcaggaatgcggtttatattatgcggcattggacaaacgatatggcattgattggcagtttatgaatgtcttcatgttgggcgtaaacggattcctattggttcagaagacaacgacgatatatttagagagaaaaagctacccagcataggataaacacacattgagcattgagagacataggtatcggtatggatgggaaaactacacacgtgaacaccaaacgacttatatactcgagcggtgatactactgagcaagaatgcactgcatctgagccactgaatgaagactgtgatgaaaatgtgaccatcgatggaattggagaagaatatgcgcagttcttcatgtccccgcaatgggtcccaaatctacatcgcttgagcgaggataccaaaaaggtataccgatgtatggtttccaacagactcaattattttccctattatgaggcgttcaggcggtctttgtttgatatgtatatgctaggtcggttggggcgtcgacttaagcgatctgactgggagactattatgcatctgtcaccaacgcaaagtcggcgtctacatagaactttaagatttgtggagcgtagaattatcccatctaacagttatatacgcacatcgggccacgttccgccttcgagggcacttccgacagatacgaatttaaagatggatgaataattaaattggaaagagtaactacattaatcgagcgtcatgacggcgtcccgtgaaaatgggaattttctactcgaaacaccgtgacatttgacagacctggaattgttattctgatatatagtgggtgtgtctggccggcaacatacataatgtgcatgcgaaaccactttttcagtgtacgctgacattgtgcaacacggaggggtagcatctacatacaatatatgttgattaatgattggagaaaaaactatgcagctcgccgatcatatggctaactcgccttcgtctatatggcggaccccgcgggaaaaatcgacgtaccatctgatttacaacaccagtaatgaacatgtcgcatccctgcccagatctgtgcgcccattggcgcggatcgttgtgaatgccgccgaaacacttcaggtcggtatgagagccgggaggccgccatcagcaggagtttggcgagaggtgtttgatagaatgatgacagccttccgtgaccacgagcctactgcgacatttaatgctgcaaatcccattagaaaaatggtcgagacagttctacagaataatgaagagcccccgcggacgcatgctgaaatgggtaatcgccttatgaacattatgtactggtgttgcttgggacacgcaggacaatgctcgatatggcagttgtacgagacgaatcaggccattttaagtttattagatgaagtggttatcggcacaacaaatcccttttgcaccctcgagcaatactggaagccattatgcaccgcaatcgccaacaaggggacctcatcgcttgttgaggatgccaaagtggccgagtacctggttagcatgcgcaaattgatataacataggcacgctctgatgttacagaccacaataccgcatacatttattgtaaggttgttaataaaggtttattctatgtaagactacaatactttcgacattgcttgtatacatattaaatactttctcaagttcctattacataaaatgggatctatcattacattcgttaagagtctggataattttactgtttgccagcttcgatcttggaacgtactgtggatagtgccttacttggaatcgtgaaaatttgaaacgtccattatttggatatcttccggttgtcccatatcccgccctggtaccgctcggataccttgcccgtatggattcgtattgacagtcgcgcaatcggggaccaacaacgcgtgggtccacactcattcggaaattttccgatgattctgaatatttattgccgctcgttacgagtcgttggacatatctgtaatacatttcttcttctgaaggatcgctgcacatttgatctatacattggccaggatgttcaagtctcagatgttgcattctggcacagcacaactttatggcatttccgatgtaatcgtccggcagccctgggggagttctatattcgcatattgggatggtaaggacaatagcagatctcgcaacctccagggaggctataataacgtttttaaaggatggatttctcataaaaatctgtcgcaaattacactgagaatatcctttactagcgccgattgagagcatcgtcgtccaattttctaaatggaaagaaaacaaggcgggcaagagtgttccaaacattttcattttcggcgaatctctcaaatcccatggcgtgcaattgattgcaaaattggcacttccgttcacgtttgtatctccaaactctaagacacttttaattgaaaaactacgttctagtgtggaaagaaacctataggcagaccatagaactatttgacaccacatatctttttgtatgtcaaactgaccatgatcgtatgttgctgaatgcactagggcaattcgctcgcgcgactccatacattgaataattccacacgtcagctcatcggttagcaaggtccagtagttgaagtcatttatttttccccgcggctggccaaatctacctctgggaatatccaagttgtcgaatatgatcgcaccggctctggtcatggtgaaggaactgtagcataaagacgcaggtatcataggggtaatatttttttattcactcacatactaaaagtaacgcatattagcaccatgtatgggctatcaattgacatttgcgtagcactacatcacgattatgtacaacataatgggacaacatatggcaagtagatgcaatttcctcacactagttgggtttatctactattgaattttcccctatctgtgatacacttgggagcctctacaagcatattgccatcatgtacgtttttatctactgtcttaacgcccatgggaacggaggcgtcgtcgtcatgtattggacggcaacataggcagcaacacaaattgcgtttaggtggggtgcatgtggactcgataccaagcccctgcagctggggaacgtctggtggagagccgataatttgatatacgcacgccatattactgtcgttgaagtacgccttatcttctatgttttcaaatttaggttcccaagtggacgtgagaagtgtttgtatctcacatggaatggcccaaggcattccagcccaggtgcctggtactttaatggcaaacaaacgttttggtagaggtattgattctattgcagttctgcagatatctgcagccccgagtatccacaggctatacgatacgttatcggaggcaagcttgttaattaagtcgacggcagagtcgcagacgcccctattggacgtcaaaattgtagaggtgaagttttcaaacgatggcgaagtaacggcgacttgcgtttccaccgtcaaatctccctatagggtagaaactaattggaaagtagacctcgtagatgtaatggatgaaatttctgggaacagtcccgccggggtttttaacagtaatgagaaatggcagaaacagctgtactacagagtaaccgatggaagaacatcggtccagctaatgtgcctgtcgtgcacgagccattctccggaaccttactgtcttttcgacacgtctcttatagcgagggaaaaagatatcgcgccagagttatactttacctctgatccgcaaacggcatactgcacaataactctgccgtccggcgttgttccgagattcgaatggagccttaataatgtttcactgccggaatatttgacggccacgaccgttgtttcgcataccgctggccaaagtacagtgtggaagagcagcgcgagagcaggcgaggcgtggatttctggccggggaggcaatatatacgaatgcaccgtcctcatctcagacggcactcgcgttactacgcgaaaggagaggtgcttaacaaacacatggattgcggtggaaaacggtgctgctcaggcgcagctgtattcactcttttctggacttgtgtcaggattatgcgggagcatatctgctttgtacgcaacgctatggaccgccatttatttttgaggaatgctttttggactatcgtactgctttcttccttcgctagccagagcaccgccgccgtcacgtacgactacattttaggccgtcgcgcgctcgacgcgctaaccataccggcggttggcccgtataacagatacctcactagggtatcaagaggctgcgacgttgtcgagctcaacccgatttctaacgtggacgacatgatatcggcggccaaagaaaaagagaaggggggccctttcgaggcctccgtcgtctggttctacgtgattaagggcgacgacggcgaggacaagtactgtccaatctatagaaaagagtacagggaatgtggcgacgtacaactgctatctgaatgcgccgttcaatctgcacagatgtgggcagtggactatgttcctagcacccttgtatcgcgaaatggcgcgggactgactatattctcccccactgctgcgctctctggccaatacttgctgaccctgaaaatcgggagatttgcgcaaacagctctcgtaactctagaagttaacgatcgctgtttaaagatcgggtcgcagcttaactttttaccgtcgaaatgctggacaacagaacagtatcagactggatttcaaggcgaacacctttatccgatcgcagacaccaatacacgacacgcggacgacgtatatcggggatacgaagatattctgcagcgctggaataatttgctgaggaaaaagaatcctagcgcgccagaccctcgtccagatagcgtcccgcaagaaattcccgctgtaaccaagaaagcggaagggcgcaccccggacgcagaaagcagcgaaaagaaggcccctccagaagactcggaggacgacatgcaggcagaggcttctggagaaaatcctgccgccctccccgaagacgacgaagtccccgaggacaccgagcacgatgatccaaactcggatcctgactattacaatgacatgcccgccgtgatcccggtggaggagactactaaaagttctaatgccgtctccatgcccatattcgcggcgttcgtagcctgcgcggtcgcgctcgtggggctactggtttggagcatcgtaaaatgcgcgcgtagctaatcgagcctagaataggtggtttcttcctacatgccacgcctcacgctcataatataaatcacatggaatagcataccaatgcctattcattgggacgttcgaaaagcatggcatcgctacttggaactctggctctccttgccgcgacgctcgcacccttcggcgcgatgggaatcgtgatcactggaaatcacgtctccgccaggattgacgacgatcacatcgtgatcgtcgcgcctcgccccgaagctacaattcaactgcagctatttttcatgcctggccagagaccccacaaaccctactcaggaaccgtccgcgtcgcgtttcggtctgatataacaaaccagtgctaccaggaacttagcgaggagcgctttgaaaattgcactcatcgatcgtcttctgtttttgtcggctgtaaagtgaccgagtacacgttctccgcctcgaacagactaaccggacctccacacccgtttaagctcactatacgaaatcctcgtccgaacgacagcgggatgttctacgtaattgttcggctagacgacaccaaagaacccattgacgtcttcgcgatccaactatcggtgtatcaattcgcgaacaccgccgcgactcgcggactctattccaaggcttcgtgtcgcaccttcggattacctaccgtccaacttgaggcctatctcaggaccgaggaaagttggcgcaactggcaagcgtacgttgccacggaggccacgacgaccagcgccgaggcgacaaccccgacgcccgtcactgcaaccagcgcctccgaacttgaagcggaacactttacctttccctggctagaaaatggcgtggatcattacgaaccgacacccgcaaacgaaaattcaaacgttactgtccgtctcgggacaatgagccctacgctaattggggtaaccgtggctgccgtcgtgagcgcaacgatcggcctcgtcattgtaatttccatcgtcaccagaaacatgtgcaccccgcaccgaaaattagacacggtctcgcaagacgacgaagaacgttcccaaactagaagggaatcgcgaaaatttggacccatggttgcgtgcgaaataaacaagggggctgaccaggatagtgaacttgtggaactggttgcgattgttaacccgtctgcgctaagctcgcccgactcaataaaaatgtgattaagtctgaatgtggctctccaatcatttcgattctctaatctcccaatcctctcaaaaggggcagtatcggacacggactgggaggggcgtacacgatagttatatggtacagcagaggcctctgaacacttaggaggagaattcagccggggagagcccctgttgagtaggcttgggagcatattgcaggatgaacatgttagtgatagttctcgcctcttgtcttgcgcgcctaacttttgcgacgcgacacgtcctctttttggaaggcactcaggctgtcctcggggaagatgatcccagaaacgttccggaagggactgtaatcaaatggacaaaagtcctgcggaacgcgtgcaagatgaaggcggccgatgtctgctcttcgcctaactattgctttcatgatttaatttacgacggaggaaagaaagactgcccgcccgcgggacccctgtctgcaaacctggtaattttactaaagcgcggcgaaagcttaggtcaattccctggcattatgcccagtacatgaccttatgggactttcctacttggcagtacatctacgtattagtcatcgctattaccatggtgatgcggttttggcagtacatcaatgggcgtggatagcggtttgactcacggggatttccaagtctccaccccattgacgtcaatgggagtttgttttggcaccaaaatcaacgggactttccaaaatgtcgtaacaactccgccccattgacgcaaatgggcggtaggcgtgtacggtgggaggtctatataagcagagctcgtttagtgaaccgtcagatcgcctggagacgccatccacgctgttttgacctccatagaagacaccgggcgcgccggatctatgacaaacctgcaagatcaaacccaacagattgttccgttcatacggagccttctgatgccaacaaccggaccggcgtccattccggacgacaccctggagaagcacactctcaggtcagagacctcgacctacaatttgactgtgggggacacagggtcagggctaattgtctttttccctggattccctggctcaattgtgggtgctcactacacactgcagagcaatgggaactacaagttcgatcagatgctcctgactgcccagaacctaccggccagctacaactactgcagactagtgagtcggagtctcacagtgaggtcaagcacactccctggtggcgtttatgcactaaacggcaccataaacgccgtgaccttccaaggaagcctgagtgaactgacagatgttagctacaatgggttgatgtctgcaacagccaacatcaacgacaaagttgggaatgtcctggtaggggaaggggtcactgtcctcagcctacccacatcatatgatcttgggtatgtgaggcttggtgaccccattcccgctatagggcttgacccaaaaatggtagctacatgcgacagcagtgacaggcccagagtctacaccataactgcagccgatgattaccaattctcatcacagtaccaaccaggtggggtaacaatcacactgttctcagccaacattgatgctatcacaagcctcagcattgggggagagctcgtgtttcaaacaagcgtccaaggccttgtactgggcgccaccatctaccttataggctttgatgggactgcggtaatcaccagagctgtggccgcagataatgggctgacggccggcaccgacaatcttatgccattcaatcttgtcattccaaccaatgagataacccagccgatcacatccatcaaactggagatagtgacctccaaaagtggtggtcaggcaggggatcagatgtcatggtcggcaagtgggagcctagcagtgacgatccatggtggcaactatccaggggccctccgtcccgtcacactagtagcctacgaaagagtggcaacaggatccgtcgttacggtcgctggggtgagtaacttcgagctgatcccaaatcctgaactagcaaagaacctggttacagaatacggccgatttgacccaggagccatgaactacacaaaattgatactgagtgagagggaccgtcttggcatcaagaccgtctggccaacaagggagtacactgattttcgtgagtacttcatggaggtggccgacctcaactctcccctgaagattgcaggagcatttggcttcaaagacataatccgggctataaggaggtaagatccataattgattgacgggagatgggggaggctaactgaaacacggaaggagacaataccggaaggaacccgcgctatgacggcaataaaaagacagaataaaacgcacgggtgttgggtcgtttgttcataaacgcggggttcggtcccagggctggcactctgtcgataccccaccgagaccccattggggccaatacgcccgcgtttcttccttttccccaccccaccccccaagttcgggtgaaggcccagggctcgcagccaacgtcggggcggcaggccctgccatagccactggccccgtgggttagggacggggtcccccatggggaatggtttatggttcgtgggggttattattttgaagcttgcctccgattctagcattacatagccggtcagtagatcctgccattcggtagcgcaaccggctacatcttcaaacagtctcacaataaatgcatctctcgttcctgccaatccggaaccgggcataccactcccgcctgccgatttaattctcacaattgggcgatgccggcggggcaaaacgaatgtggatttggcaaaccgacacaggtctgctgtacggactaatatgggcacacccacatcattcttcagatgctccatgcattgttctatgagaaagatccatagggtggaggcagcgtcacgagatcgcccaggcaatcgatcgcattcgtctagtaaagtgacgagagttatcatgcacacacccatgcccacgccttccgaataactggagctgtggaagatcggaaacgtctttttgactgccggtctcgtactactttcgcacaggtgtatacccggacgcgtactatatattttatatcatccaacgtccgaaattacatacgtggcggcgatggaagtagatgttgagtcttcgaaagtaagtgcctcgaatatgggtattgtctgtgaaaatatcgaaagcggtacgacggttgcagaaccgtcgatgtcgccagatactagtaacaatagcttcgataacgaagacttccgtgggcctgaatacgatgtggagataaataccagaaaatctgctaatcttgatcgtatggaatcttcgtgccgtgaacaacgagcggcgtgcgaacttcgaaagtgttcgtgtcctacgtctgccgtgcgcatgcaatacagtattctttcatctctcgctccgggttcagagggtcatgtatatatatgtactagatacggggacgcggaccaaaaaaaatgcatagtgaaggcagtcgttggaggaaagaatcccgggagggaagtggatattttaaaaaccatctcacataaatcaattataaaattaatccatgcctataaatggaaaaatgttgtgtgtatggcaatgcgtgtatatcgttatgatcttttcacatatattgacggagtcggccctatgccccttcaacagatgatctatattcaacgtggactactagaggcgctagcatacatacatgaaaggggcatcattcaccgagacgtaaagacggagaatatattcttggataatcacgaaaatgcagttttgggtgacttcggtgctgcatgccaactaggagattgtatagatacgccccaatgttacggttggagcggaactgtggaaacaaattcgccggaattatctgcacttgatccgtattgcacaaaaacagatatttggagtgccggattggttctatatgagatggcaattaaaaatgtaccattgtttagtaagcaggtgaaaagttcgggatctcagctgagatccataatacggtgcatgcaagtgcatgaactggagtttccccgcaacgattctaccaacctctgtaaacatttcaaacaatatgcggttcgtgtacgaccgccttataccattcctcgagttataagaaatggggggatgccaatggatgttgaatatgtcatttctaaaatgcttacgtttgaccaggagttcagaccttctgctaaggaaatattgaatatgcccctatttactaaggcgccgattaacctgcttaatatcacaccctctgacagtgtctaacggtatacaggcgggagcgggtcgtggcgtcatcatcaccacttgagaatttatattttgaattgttgattgataaattaacctgattcattgagaactgaaacgccatattggtttcttggatatgtctacaacaattagttaaattgctatgttctactgcgagtaacatttgataagttgtaagagacgggcgactcatgtcgaagttgacgaatataaagtacataacgtgtttagaatacccagaatccgaatagtccgcgggggcgtcttctcgcgtgagtaccaaatactgagttgaacttgaaaatgctaaatctgtgacactctttgtgtgatgattattgtcaccacttcgaagatggcttcgacattcatgatgttctggtgtttgtttggaatcgtaatagcgcttgtttcgtccaagtctgacaacaaagaaaatctgaagaattatatcacggataagtcaaccaatattagaatacccacgccattatttgtatcaacggaaaactcttatcccacaaaacatgtaatctacgatgaaaactgtggcttcgctgtactcaatcctataagtgaccccaaatatgtccttttgagccagcttctaatgggaaggcgcaaatatgatgcgacggtcgcgtggtttgttctcggtaaaatgtgtgccagattaatatatttgcgcgaattttataactgctcgacaaatgagccttttggcacatgttctatgagctctcctggatggtgggacaggcgctacgtctcaaccagtttcatttctcgcgacgaattacagctggtttttgcagcgccgtcccgagaattagatggtttatatacgcgcgtagtagttgtcaacggggactttactacggccgatataatgtttaatgttaaagtggcatgtgccttttcaaagactggaatagaagatgatacattatgcaaaccctttcatttctttgccaatgcaacattgcacaatttaaccatgattagatcggtaactcttcgagcgcacgaaagccatttaaaggaatgggtggcacggagaggtggtaacgtccctgcagtgctacttgagtctaccatgtatcatgcatccaatctgcctagaaatttcagggatttctacataaagtctccagatgattataagtataatcacctagatgggccatctgtaatgctcatcactgacagacctagtgaagatttggatgggaggctcgttcaccaaagtgacatttttactactacaagtcctataaaacaggtccggtatgaagagcatcagtcacatacaaagcagtatcctgtaaacaaaatacaagctataatttttttgatagggttaggctcgttcattggaagcatattcgtagttttggtagtatggattatacgcagatattgcaatggagcgcggagtgggggaacgccccccagtcctcgccggtatgtgtataccaggctatgatcacgtgtgaaacttgggcggacctgtatcatatgtacaccgtccctattcgtttatagccagtacgtgttatctgcacatagaggaacatgtgtcatactgggatcgcatgcatggtatgtgtgactctaatattattctgtatcataataaaaacacagtgcatggtatatagaggatcgctggtaagcactacggtagaccaatcggctcagattgcattctttggcatcgataccgttgttaatttatatggcaaagtcttgttcatgggagatcagtatttggaggaaatatactctggaacgatggaaatactcaaatggaatcaagctaaccgctgctattctattgcgcatgcaacatattacgccgactgtcctataatcagttctacggtattcagaggatgccgggacgccgttgtttatactaggccccacagcagaattc

SEQ ID NO: 18 - DNA, 15252 bp, synthetic construct
  misc_feature 1..15252: note = Herpesvirus of turkeys, murine cytomegalovirus, Infectious bursal disease virus, Simian vacuolating virus 40, and Infectious laryngotracheitis virus
  source 1..15252: mol_type = other DNA
ggcgcgccactggagaacggcatgaccgcaaaaggcgttgtagagatcgatcccacgaactctcaggcgatcgtgtcagtcgccataaacagcgacgatcgtctccaggatctgaacggttttcttctcaacgatcatcagtatatgaggaactgaacctgatatttagccgagggaaacgcaggttaaaaaccctatcaagcgattgcgattttcgcgtatctagtaaaaatagatgggcttcggtactagccttcgccgccaactctgaatatgcccttcgtggacctcatataacatggcattgtttgttggatgcggggccggaattaagaagaacattcgaaatacgagcaaaaatttcggccctggcatgtgctgcgcgagaatcggtacttcggggagaaagttttatcggagctttgggtagtgcagaggaaactctatcttggttgaaaatgcatgcgaccctgcacttgattctggttaaccacgatccaatttttaagacggctggcgcggtcctagataacctccgcttaaaactagccccaatattgatgtgcagatataacacagaaaaacgatcaatggaagacatgctacggcggtcatctcccgaagacatcaccgattccctaacaatgtgcctgattatgttatcgcgcattcgtcgtaccatgcgcaccgcaggaaataaatatagctatatgatagatccaatgaatcgtatgtctaattacactccaggcgaatgtatgacaggtatattgcgatatattgacgaacatgctagaaggtgtcctgatcacatatgtaatttgtatatcacatgtacacttatgccgatgtatgtgcacgggcgatatttctattgtaattcatttttttgttagtaaactaccacaggctgtccggaaatctaagttaatgaataaagtagatggttaatactcattgcttagaattggactacttttaattctctttaatgttcgtattaaataaaaacatctttaataaacttcagcctcttcgcttattgtagaaattgagtattcaaaatcatgttcaaagccgtcttcggagagtgtactcgccacggtggttggaacatcactatgtctacacgtcaaatttaagcacgtcaggtctgtcgaggacaagaaatggttaactagtgtttcaattattcttataaacgttaagcattgtaagccccccggccgtccgcagcaacaatttactagtatgccgtgggctccgggactatcacggatgtccaattcgcacatgcatataatttttctagggtctctcatttcgagaaatcttcggggatccatcagcaatgcgggctgtagtcccgattcccgtttcaaatgaaggtgctccaacacggtcttcaaagcaaccggcataccagcaaacacagactgcaactccccgctgcaatgattggttataaacagtaatctgtcttctggaagtatatttcgcccgacaatccacggcgcccccaaagttaaaaaccatccatgtgtatttgcgtcttctctgttaaaagaatattgactggcattttcccgttgaccgccagatatccaaagtacagcacgatgttgcacggacgactttgcagtcaccagccttcctttccacccccccaccaacaaaatgtttatcgtaggacccatatccgtaataaggatgggtctggcagcaaccccataggcgcctcggcgtggtagttctcgaggccttaagcttaaggatcccccaactccgcccgttttatgactagaaccaatagtttttaatgccaaatgcactgaaatcccctaatttgcaaagccaaacgccccctatgtgagtaatacggggactttttacccaatttcccacgcggaaagccccctaatacactcatatggcatatgaatcagcacggtcatgcactctaatggcggcccatagggactttccacatagggggcgttcaccatttcccagcataggggtggtgactcaatggcctttacccaagtacattgggtcaatgggaggtaagccaatgggtttttcccattactggcaagcacactgagtcaaatgggactttccactgggttttgcccaagtacattgggtcaatgggaggtgagccaatgggaaaaacccattgctgccaagtacactgactcaatagggactttccaatgggtttttccattgttggcaagcatataaggtcaatgtgggtgagtcaatagggactttccattgtattctgcccagtacataaggtcaatagggggtgaatcaacaggaaagtcccattggagccaagtacactgcgtcaatagggactttccattgggttttgcccagtacataaggtcaataggggatgagtcaatgggaaaaacccattggagccaagtacactgactcaatagggactttccattgggttttgcccagtacataaggtcaatagggggtgagtcaacaggaaagttccattggagccaagtacattgagtcaatagggactttccaatgggttttgcccagtacataaggtcaatgggaggtaagccaatgggtttttcccattactggcacgtatactgagtcattagggactttccaatgggttttgcccagtacataaggtcaataggggtgaatcaacaggaaagtcccattggagccaagtacactgagtcaatagggactttccattgggttttgcccagtacaaaaggtcaatagggggtgagtcaatgggtttttcccattattggcacgtacataaggtcaataggggtgagtcattgggtttttccagccaatttaattaaaacgccatgtactttcccaccattgacgtcaatgggctattgaaactaatgcaacgtgacctttaaacggtactttcccatagctgattaatgggaaagtaccgttctcgagccaatacacgtcaatgggaagtgaaagggcagccaaaacgtaacaccgccccggttttcccctggaaattccatattggcacgcattctattggctgagctgcgttctacgtgggtataagaggcgcgaccagcgtcggtaccgtcgcagtcttcggtctgaccaccgtagaacgcagagctcctcgctgcaggcggccgctctagaactcgtcgatcgcagcgatgacaaacctgcaagatcaaacccaacagattgttccgttcatacggagccttctgatgccaacaaccggaccggcgtccattccggacgacaccctggagaagcacactctcaggtcagagacctcgacctacaatttgactgtgggggacacagggtcagggctaattgtctttttccctggattccctggctcaattgtgggtgctcactacacactgcagagcaatgggaactacaagttcgatcagatgctcctgactgcccagaacctaccggccagctacaactactgcagactagtgagtcggagtctcacagtgaggtcaagcacactccctggtggcgtttatgcactaaacggcaccataaacgccgtgaccttccaaggaagcctgagtgaactgacagatgttagctacaatgggttgatgtctgcaacagccaacatcaacgacaaaattgggaatgtcctggtaggggaaggggtcactgtcctcagcctacccacatcatatgatcttgggtatgtgaggcttggtgaccccattcccgctatagggcttgacccaaaaatggtagctacatgcgacagcagtgacaggcccagagtctacaccataactgcagccgatgattaccaattctcatcacagtaccaaccaggtggggtaacaatcacactgttctcagccaacattgatgctatcacaagcctcagcattgggggagagctcgtgtttcaaacaagcgtccaaggccttgtactgggcgccaccatctaccttataggctttgatgggactgcggtaatcaccagagctgtggccgcagataatgggctgacggccggcaccgacaatcttatgccattcaatcttgtcattccaaccaatgagataacccagccaatcacatccatcaaactggagatagtgacctccaaaagtggtggtcaggcaggggatcagatgtcatggtcggcaagtgggagcctagcagtgacgatccatggtggcaactatccaggggccctccgtcccgtcacactagtagcctacgaaagagtggcaacaggatccgtcgttacggtcgctggggtgagtaacttcgagctgattccaaatcctgaactagcaaagaacctggttacagaatacggccgatttgacccaggagccatgaactacacaaaattgatactgagtgagagggaccgtcttggcatcaagaccgtctggccaacaagggagtacactgattttcgtgagtacttcatggaggtggccgacctcaactctcccctgaagattgcaggagcatttggcttcaaagacataatccgggctataaggaggtagatccagacatgataagatacattgatgagtttggacaaaccacaactagaatgcagtgaaaaaaatgctttatttgtgaaatttgtgatgctattgctttatttgtaaccattataagctgcaataaacaagttaacaacaacaattgcattcattttatgtttcaggttcagggggaggtgtgggaggttttttcggatcctctagagtcgacggcagagtcgcagacgcccctattggacgtcaaaattgtagaggtgaagttttcaaacgatggcgaagtaacggcgacttgcgtttccaccgtcaaatctccctatagggtagaaactaattggaaagtagacctcgtagatgtaatggatgaaatttctgggaacagtcccgccggggtttttaacagtaatgagaaatggcagaaacagctgtactacagagtaaccgatggaagaacatcggtccagctaatgtgcctgtcgtgcacgagccattctccggaaccttactgtcttttcgacacgtctcttatagcgagggaaaaagatatcgcgccagagttatactttacctctgatccgcaaacggcatactgcacaataactctgccgtccggcgttgttccgagattcgaatggagccttaataatgtttcactgccggaatatttgacggccacgaccgttgtttcgcataccgctggccaaagtacagtgtggaagagcagcgcgagagcaggcgaggcgtggatttctggccggggaggcaatatatacgaatgcaccgtcctcatctcagacggcactcgcgttactacgcgaaaggagaggtgcttaacaaacacatggattgcggtggaaaacggtgctgctcaggcgcagctgtattcactcttttctggacttgtgtcaggattatgcgggagcatatctgctttgtacgcaacgctatggaccgccatttatttttgaggaatgctttttggactatcgtactgctttcttccttcgctagccagagcaccgccgccgtcacgtacgactacattttaggccgtcgcgcgctcgacgcgctaaccataccggcggttggcccgtataacagatacctcactagggtatcaagaggctgcgacgttgtcgagctcaacccgatttctaacgtggacgacatgatatcggcggccaaagaaaaagagaaggggggccctttcgaggcctccgtcgtctggttctacgtgattaagggcgacgacggcgaggacaagtactgtccaatctatagaaaagagtacagggaatgtggcgacgtacaactgctatctgaatgcgccgttcaatctgcacagatgtgggcagtggactatgttcctagcacccttgtatcgcgaaatggcgcgggactgactatattctcccccactgctgcgctctctggccaatacttgctgaccctgaaaatcgggagatttgcgcaaacagctctcgtaactctagaagttaacgatcgctgtttaaagatcgggtcgcagcttaactttttaccgtcgaaatgctggacaacagaacagtatcagactggatttcaaggcgaacacctttatccgatcgcagacaccaatacacgacacgcggacgacgtatatcggggatacgaagatattctgcagcgctggaataatttgctgaggaaaaagaatcctagcgcgccagaccctcgtccagatagcgtcccgcaagaaattcccgctgtaaccaagaaagcggaagggcgcaccccggacgcagaaagcagcgaaaagaaggcccctccagaagactcggaggacgacatgcaggcagaggcttctggagaaaatcctgccgccctccccgaagacgacgaagtccccgaggacaccgagcacgatgatccaaactcggatcctgactattacaatgacatgcccgccgtgatcccggtggaggagactactaaaagttctaatgccgtctccatgcccatattcgcggcgttcgtagcctgcgcggtcgcgctcgtggggctactggtttggagcatcgtaaaatgcgcgcgtagctaatcgagcctagaataggtggtttcttcctacatgccacgcctcacgctcataatataaatcacatggaatagcataccaatgcctattcattgggacgttcgaaaagcatggcatcgctacttggaactctggctctccttgccgcgacgctcgcacccttcggcgcgatgggaatcgtgatcactggaaatcacgtctccgccaggattgacgacgatcacatcgtgatcgtcgcgcctcgccccgaagctacaattcaactgcagctatttttcatgcctggccagagaccccacaaaccctactcaggaaccgtccgcgtcgcgtttcggtctgatataacaaaccagtgctaccaggaacttagcgaggagcgctttgaaaattgcactcatcgatcgtcttctgtttttgtcggctgtaaagtgaccgagtacacgttctccgcctcgaacagactaaccggacctccacacccgtttaagctcactatacgaaatcctcgtccgaacgacagcgggatgttctacgtaattgttcggctagacgacaccaaagaacccattgacgtcttcgcgatccaactatcggtgtatcaattcgcgaacaccgccgcgactcgcggactctattccaaggcttcgtgtcgcaccttcggattacctaccgtccaacttgaggcctatctcaggaccgaggaaagttggcgcaactggcaagcgtacgttgccacggaggccacgacgaccagcgccgaggcgacaaccccgacgcccgtcactgcaaccagcgcctccgaacttgaagcggaacactttacctttccctggctagaaaatggcgtggatcattacgaaccgacacccgcaaacgaaaattcaaacgttactgtccgtctcgggacaatgagccctacgctaattggggtaaccgtggctgccgtcgtgagcgcaacgatcggcctcgtcattgtaatttccatcgtcaccagaaacatgtgcaccccgcaccgaaaattagacacggtctcgcaagacgacgaagaacgttcccaaactagaagggaatcgcgaaaatttggacccatggttgcgtgcgaaataaacaagggggctgaccaggatagtgaacttgtggaactggttgcgattgttaacccgtctgcgctaagctcgcccgactcaataaaaatgtgattaagtctgaatgtggctctccaatcatttcgattctctaatctcccaatcctctcaaaaggggcagtatcggacacggactgggaggggcgtacacgatagttatatggtacagcagaggcctctgaacacttaggaggagaattcagccggggagagcccctgttgagtaggcttgggagcatattgcaggatgaacatgttagtgatagttctcgcctcttgtcttgcgcgcctaacttttgcgacgcgacacgtcctctttttggaaggcactcaggctgtcctcggggaagatgatcccagaaacgttccggaagggactgtaatcaaatggacaaaagtcctgcggaacgcgtgcaagatgaaggcggccgatgtctgctcttcgcctaactattgctttcatgatttaatttacgacggaggaaagaaagactgcccgcccgcgggacccctgtctgcaaacctggtaattttactaaagcgcggcgaaagcttcccgggttaattaaggccctcgaggatacatccaaagaggttgagtattctctctacacttcttgttaaatggaaagtgcatttgcttgttcttacaatcggcccgagtctcgttcacagcgcctcgttcacacttaaaccacaaatagtctacaggctatatgggagccagactgaaactcacatatgactaatattcgggggtgttagtcacgtgtagcccattgtgtgcatataacgatgttggacgcgtccttattcgcggtgtacttgatactatggcagcgagcatgggatattcatcctcgtcatcgttaacatctctacgggttcagaatgtttggcatgtcgtcgatcctttgcccatcgttgcaaattacaagtccgatcgccatgaccgcgataagcctgtaccatgtggcattagggtgacatctcgatcatacattataagaccaacgtgcgagtcttccaaagacctgcacgccttcttcttcggattgtcaacgggttcttcagaatctatgcccatatctggcgttgagaccattgtgcgtttaatgaacaataaagcggcatgccatggaaaggagggctgcagatctccattttctcacgccactatcctggacgctgtagacgataattataccatgaatatagagggggtatgtttccactgccactgtgatgataagttttctccagattgttggatatctgcattttctgctgccgaacaaacttcatcgctatgcaaagagatgcgtgtgtacacgcgccggtggagtatacgggaaactaaatgttcatagaggtctttgggctatatgttattaaataaaataattgaccagtgaacaatttgtttaatgttagtttattcaatgcattggttgcaaatattcattacttctccaatcccaggtcattctttagcgagatgatgttatgacattgctgtgaaaattactacaggatatatttttaagatgcaggagtaacaatgtgcatagtaggcgtagttatcgcagacgtgcaacgcttcgcatttgagttaccgaagtgcccaacagtgctgcggttatggtttatgcgcacagaatccatgcatgtcctaattgaaccatccgatttttcttttaatcgcgatcgatgtttgggcaactgcgttatttcagatctaaaaaatttaccctttatgaccatcacatctctctggctcataccccgcttggataagatatcatgtagattccgccctaagaaatgcaaactaacattattgtcggttccatatacacttccatcttgtccttcgaaaataacaaactcgcgcaatagaccgtccgtacatgcatggccgatgtgtgtcaacatcattggtctgctagatcccgatgggacgaatcgtacagtcgtcgctccagcattggcaaaaatccccagataccctccatgcggcaaatctaaattgcgaccccgaagagactgcaccaaagtcttatcgacgcacgctgatttttttgaacagcgggagcccattatcttcagtggagcgtagacgggcgaggctaattatgtgacatagcaacactgcatgtatgtttttataaatcaataagagtacataatttattacgtatcatttccgtttgtaatatactgtatacatcatccacactattagtcagcactagcgcgcgggcgcacgttacaatagcagcgtgcccgttatctatattgtccgatatttacacataacatttcatcgacatgattaaatacctaagtactgcacacagatgtttaatgtatatcgtcatataaattatatcgctaggacagacccaaacgacctttatcccaaacagtcagatcctcttctcaagtgtcgatttctgttatggaatatgcataccctggcccagaaattgcacgcacgagcgtagtgaatgcgtcattggttttacatttaaaggctaaatgcacaaattctttagacgacagcacatcgttaaatagcatctctagcgttcttatgaatgctaagcattggagtcctcctggtcggccacaataacagctgagtatcataccctgagctccggggttgtcgcacatagcggattcgtataaacataggattttccgcgaatccatcagttgcaaaaatctgttaggctccatcaacaacgctggatttacttcagatccacgcgtaaagtaatggtgctcgaataccgtttttagagttgtcggcatttcaaggaacaaagaattcatttcttcattgcaacgacgcgccagaaatcccaagacctctttgggtagtatgttcttgcctataaaacacggcgttccaagtgccaggaaccacgcatgtgttactgttggggcgtattcagaaataaagcggggtttatgcggcttttgaagctcggatatccaaagtatcgcttgctgatgaacgagcgatgtagctgttacaaaacctcctttccatcctccagtcaacataatatttatcggcctacctatgtccgtaataagtattggtcgggcaattattccgtatgaggtcttgcaggaataagctcttagggacagccagcttggatatggtgcgaaacagaccttctcggcttcagaatgtcgctccgcagtctcttcgtgtcggtgcatcttagatccaccatcaatgtgtgcagcattgactcccgcccgtcgaatattccttttgttacgatgcagtaatgagcacgatcatgggcggggcgatgacgttctatttgcatgtctgcgaacaatttgcgtcagtcatacagctatggagtgggccatttctggccgtcaacttaaaaacgcgaaccgcagacatatgtatttgcatgcaaagacgtatcttcgtatttctgggcatcttcaaatgctctggccaatatggcaatgaatttggattcgtttgacgccgatggtatgcagtgcaaatgtgccaatagcccacatccgaaaaagttatttgtcatacaagcaggtgttaagtagcaatcacataaaggcaccagacgcctcatggcatcataatgaatagctccttctccccactggaaccactgacaaaatctgcgagtatattccgcaaaccacattttatttctcatagaaactaccctaaatccttttaacgggaagaagaatcctagatagtgcttgaagtcatgactgttactgctgcaataacactgtatattatttataaattccgtttgtctaggtatctgatgtaggcattccgatccctttactattgcgtcttcacgaccaaatgggaatgcgccaaaatccccacacctcatcaccctggaggcagattgtgtattattaatatccgccgattgaagcacaaaacggtacggtactgttcctaattctggtatagattctatggtcaaaagtctgcatatccccgacattgccatgagatcacacagtccaagtagcatgtttattgagtcactcagactgtcaacgtccctcgccgcaccaccaatcgaaaataaagtatctacgcaagttatagctccgcattttctatcgctagcagcaatcgcgacgcaaaacataaaggccatgttgggatttgaactctctggggggcttgttatcttctgcaccgtcgcagtcgcagttttccgaaatttatgtctaatatattttccggccgtgctccaatcggccgaaaagaatctgcgtattaccagactcattgacgggccgataaagaccataaaacaaaattcctgtgcactccctcctccagttttgccatcgtccaagtcccgtaactttttttgcgtttcgaggagcaagcgttcgttatccctacccacacttgttttccaccgttttcttattataagcggttgtatcgccaacgcgtcaccgcaggttgtcacatacagtgatggcatacttgaacgtgcaacaacgcgctcgctttgcaaatctaagtcattgaccatcaaatcgcgttgagaggatagccaggcatcttttttcctagtatggtgacggtgcagccaccccaactcagttcttgtaaaaaaagctattggcgggaatttatgttctgaggtgcattctatatttatgagtccatcaaatgccattaaccagattcgtattttttcgctcgacccggcatcactatggatacaatacctttctatggcccatttcagctctcgaaccaaccacacggacaattgactaacataagtatgatctttatcacagtcgcacccatctgagttatatttatggcatccgagcgctcttactgtacggtcggatacacccatggtttttcctttatatagtcgggttatagtctgtcgggtttggcggtagcacggagtagtttgatttttaagaatcgaaaaccggcttggagagaccactgtcgaatatttgtccgtatactctacacgtgagtgttgtccattcctaggtatattcatctgttcggataccttcaattgctgttcaggcataaccttaaagcatatgttatgttgtacatcaaaacttggtgagttatgttcgattgccgcgcataaagaatcgtacatgagcgtttctgctaacatactatctatattctcacacgcccctgcatatactgttcctattccaaattcacgttttgccccatcggctatctgctcccaaaaagttgtaatataggtgccgctgggtgcgaaattttcatcagttgtattcctgataaactgaatcactttacataatttttgccacatatctgcgtgcagccatagtatcgaacccgtgggctcggagacgacagtgcgtacaatgggtattttacctttccccaacaaaataatggtatacaagttaggtccgtacctagaccttaatgtttccaattcttctgaatcactgcactctcgtaggggagtaacggtaataatttcgtctctgagccccgttttgcgttgaaaactaatcacattagataatgtgcaatcggtttcttttatccggatacatctaagtattatgacatcggtggtcattgtttccatcaacgaccatcttttacgatcgcccatactactcatggacgttgtcggtgttgaaaaatcaccagaattgcaacggatctctgggtaccatgctgctgatggaattggcggttttaattgttgtttcagtctattattgctatctttggcggggttgaataatgtggggggagagtgattgcaggaatccgaatgggtcaataaaacgaccgtgctccgttctgccggcgccgatccgattgaagctatatacttcgcttctctccccacttttccaatttgatccggaaataaaacggccccggacaacagtatcgtacgatccggatccggatcctgcttgcctacagaagaatcaacatctcgccccaatattctggtcaaaactggctcgctcatggcaacgcggacgtttcccccggtggccagtcttaatggttaatgttcttttcggcaatcttatacatcagcgggttgcgtgaatactggtcacagttcagtcatttactacacaccagcaatacgacgacggacagtaccgtcccgacgaacgcgacgcccaaaattgctatcgcgaccgcgtccgaggcgatgtcgtacgggcggtgcggggttggatcctcggcaaagagatcctcgtaattcggcggtgggagcggagggtaaagacgcgggtggggatctccctccggaccgcgcgccgggcgcggttcgaaaatgctttccgcctcgctcagtgtcaacgccaagtattcgggcgggctgggggccggaatatctcccgcgacttcttctatcggcgcggaattggagtcgcggtcgtggcgcgcttctagcgtcgtcaacggaagtccattttcggggtctcccggtgggcgttcagcgtccatcgtcgtatatgctctaacacacgtctcgctatattaaaaaaaagaagagtatcggtcagtgtcgagtgtcgccgacaatgtcgcgagttctcggcgatttaatttttggaactgctccctatgaatcccgtaactgtagcgcccgcgcagaaagccgccatcagaccaactacgtgtctgttcgatgtttgcccgccgatcgctttaccgattaaggttccggcgagaaatgacatgctcgatccaagaacaaagtttttcgcggtaaacaacaacatagttaccgtgcgagatggagaaaccacatctcccgaattagtagaggaaagcccgcgctgtcggtttggggacatatcgatcttttttgtgtttttcctaggacccttttgccagatcgtacaaagtcgcgtcttatgagcggacgttcttactgcagctcggtaggagtggggcagggttagatttcgtcggcgtttcggcccccgtatgcgccgcgccaccctcttcgccgagctctttatgcgcggtgggggtgagcgcttccggagttgcgatctccgatctcgagccgcagcccggcggtgtctctttcagtggagcgttagcgccatcatgtggttcgtggcggtggaaaggctattatgtgttaggggagagaccacgtgatcggcatgcaaatgagcaaggcgaacgcgtcagcgttcgcactgcgaaccaataatatatatattatactattggctttaggtgcgaacgtccggctagtccaatagcggggtcgcgtttcgtaccacgtgttatagaccgccctaaactcgcactcgggggtccggccgcgcccagacagggcggagacgtgccacaggggctttaaaacaccgcttcgggcaccgttcatctcggcgcgcc

SEQ ID NO: 19 - DNA, 199 bp, Simian virus 40
  source 1..199: mol_type = genomic DNA
agcttcagacatgataagatacattgatgagtttggacaaaccacaactagaatgcagtgaaaaaaatgctttatttgtgaaatttgtgatgctattgctttatttgtaaccattataagctgcaataaacaagttaacaacaacaattgcattcattttatgtttcaggttcagggggaggtgtgggaggttttttcg